European Patent Specification EP 3 585 158 B1, published July 5, 2023. Title: NON-HUMAN ANIMAL MODELS OF RETINOSCHISIS. Applicant: Regeneron Pharmaceuticals, Inc. The sequence listing filed with the application follows.

SEQUENCE LISTING (59 sequences)

SEQ ID NO: 1 - DNA, 5855 bp, Mus musculus
aacaatacctccccagactgcttgttgaggcaggggactatgtggcttaattggatgggggctgagtgaaagacctaagaactaaatgaaataagatgcttaagttaatcgcctgctcctatgccagctctccacttcacttagatcttgctgtgaccaaggacaaggagaaaatgccacacaagattgaaggcttcttcttgttacttctctttggctatgaagccacattgggattgtcatcgacagaggatgagggtgaggacccctggtaccagaaagcatgcaagtgtgattgccaggtaggagccaatgctctgtggtctgctggagctacctccttagactgtattccagaatgcccatatcacaagcccctgggtttcgagtcaggggaggtcacgccagatcagatcacttgctccaacccagagcagtatgtgggctggtattcctcatggacagcaaacaaggcccgactcaacagtcaaggttttgggtgtgcttggctttccaagtatcaggacagcagccagtggttacagatagatttgaaggagatcaaggtgatttcggggatcctgacccaaggacgctgtgacatagacgagtgggtgaccaagtacagtgtgcagtataggactgatgagcgcctgaactggatctactataaggatcagaccggaaacaatcgggtcttctatggaaactcagaccggagttctacagttcagaacttactcaggccccccatcatttcccgcttcatccgactgatccctctaggctggcatgtccgaattgccatccggatggagctgcttgagtgtgccagcaagtgtgcctgatgtctatttcagctcagttctgtcacttgcagggagagctttggggggagggcaccctgaaataccactgggatgaatggggctatatcttataagcactttacaatgtagatctgggtagagaatatttcactttttaaaagatagtttcaaatttcaaagggagagagagagagagagagagagagagagagagagagagagaagcttttaagcttttcttcaactcagggccaaagaaaataagaacaaagaaagtatctctcaaaccaattttcttacacaaacccaaatagcaggggtaatttgctgctctggctccccatctttttctctttgtctcagtgacaccgtcaaaggtgcaggcccaggggaacacaaagcagctctgataatttgaaaattctttttggctcttagcacattcagaagaggagcgtactctttggcaaagcctcacatgaacacttgcatgaaatcctcactatagaggcctggtgacaagtacataggtgtgaagaaagcagaaggaagcctggcgtatggcccacgagtctggagccagtaaccaaccaaccaactaaccaactaaccaaccagtcaaggcttccccctccctggaattgcttttgcctggaaggggtggagctccttgtgcagaaactccattctacagcccttttggcaatgtgtccttctgtgattgcctggagatgaatgcaaggggcaggctatatgtgtgtgtggatagtgaggtttcccttaaactgaggaagcccaaataactagaatacatcacaccttctttatccatggctacagtttcccagaaattgaacaggcttagaaaacagctgagataaaccatatctctatctactgggaagagatcatgctttgggggaaggggttaggactcctatcatagaggactgtacacagatgatctgtcagtaaagggcttgctgtacagcataggaacttgagattatatttctagaatgcatgtaaaaagctaggtatggacaggtatggtggaacatgccattagtcttagtatttggaagacagaggcaagcagatctgagttcagggccagcctggtctacatagcagttccaagctagccaaggctacacagtaaggccctgtttcaagaaaaaaagaccaggcatggaggggcacacctgcaaatccaggactaggaggcaggcagagacaggatgatgcctagagcttgtctgccaatcagtacactccaggttcatggtcagaccctgtctcaaaactaaagtgaagagctattgaggaagataccagatgtcaacctctgtccaacatgcacacatacacatacactggtaggtttcaaacctggggcaaatggcagaggtgcctagttaaggttctcccagcatctctcagcccctaccaggtcctcctagttggcataccccgccccctaccccgaaactcttcagcccagggggttgggcttcttccctatataatccaactattttggtcaccctttctctttgtacctttgggcctcctggttgctgcatctggttcctctgttctcccttatctcttttcctccctcctctcctcacaaggcccagcttagagtgttcatgtctattctggactctctcccggatgcccctgcctctggctatgctctcccacatatctaccataaactctctcctctaccatacctaggacaagtcatgttcctttccttttcctttttgtttcccattcaaacatgtaaataggaaaaacaaaatacaacaacaacaaacaaaaataaaaccacaaaagccttctctccgagcggcttcctcccgtcctgcccacccaaacatgcttactcagacatgacatttgaaacttctttcggtagtcattctctggcaggaatagctcatttaatcaggagctttggagcctgagagaatgactactggtctctagctcatttccatctgtagctcaagctgggtttgaggctcttctctgggagaggctgttaactggagtgagggtcaaaaaggcatgcggggagaagctgagaatgagaactgcccagagacaaggtcttggcctcacacacacacaatacagccttggttagtacttttctctgagctattttctatttccaggtattaaaggagattacatggattcacaccaaaataactttggatggccagacatggtatcttccatctttaatcctagcactgggaaaacacagacaggtggatctctgtgagttcaaggccaggtttgcatagcaagctccagaccagccaaggctatgtagtgagactgtctcaaaaatcaatccatcaatcaaatgatcttggatgtcacattcttctcagtgaatagaacaacattttaatagcatcaaatttcctacctagtattttggagttccacaggtgtgtgtgtatgtgtggcaatgtacaacaatattcctggtatgactacatatgtacaaattcattttggataatattcctgacagcagacctttatttggaaaattgagttacctttctcaccacactgagtaattgttagagaaaaatggcaataacttaagaatactgatcagggagaaaaaaacccaaatggtacaaggcatgggtaaatagtcatcaaattaaaaaatcatgccataaatttgttttctaatagtttcattaacttcacataaacagtcctaattcatttaaggtgtgtaattcaatatagtatattcaaacttgaacaatcatcactacaagtaactttagactattcttatcacccccaagagaatcctctaacaatgggccatcagccaccacagctctagattactcgtcatccattttctatttgtgtgtggattttttttccattctgggcatttctccacacaaatggaatcttagaatatatagtagtttatgacttgtttcttgtacttatcatagtgtttttaaagtccatgtgttggagaagtacatcctccttttttgttattaacattctgtgtagggtattgtattattatttatccatgcatttgggtggggctagtatgaataatgctgcttcatgaaaatttatatgtaagttattgcgtggacatgttttatcttgggcatactcacactgagaatagagaattgttgggtctcttgggaactatttctccaggtggctgtaccatcttctgttcccaccagcaatgtctaatgcttccagcctctcatctttagcaatgcttcttgtatttcattagatctgtcctagtatgtatgaagtagcattcgatgatgaatttgatttgcatttctctaataaccaatgttttttgagcatcttttcaagtcaccagtgacatatttttggagaaagttctattcagacccttgcccatataaagatttcatttcacggattcattaagagttctttgggtgttctacatacaattctcttatgcaaacatttcttccatcctgtttttcttcttgtcattgtcttggtttagttttgcaccaggatttcactatgtagctcaggctggcctggaacttgcaaagatccttctgtctctgcctcccaggttctgagattctgggtatttgccaccacacctggcctttctctgaagcacaacaaataccaaattttaatgaagtccaaccttccggtttccttttttggtgtattatctgagaaactactgtcaaaccatggtcaagaagattcactcttgtgttttcttctaaatgttttgaaaaaaaatttttaaaaagttttaaagttttaactcttactttgtgaacagttataaagtaagggtgtaatttcattctttggatatcaatatgcagctgtcttggtagcttgtgttgtcttcaccacagtcaatggtctttattcttccaaaaacaactgaccaagaatattagagtatatgctaggcctcataattctattaccacatagtcttcattactgtagcattgtagtgagttgtggaattaggacatataaatcttccaattctggttatgtttcaagactgaactaactattctgggttccttaaacttctaagtaagtatatctgtaaataagccagccaggggtctcacaatggaaaatgttttcaatttcaaaattaaataaacaatgagatattaagatctgcaagatatttatctgtagttaattttctttcaatagttaatgaaaatgttagcattttcttccttttgtgttaggatatatatataaaagaaaccctattattaaagtaaacctgaaaaagaatcttcctattaaacaaaaaatatgtttgcaatattatttcttttagggggcaactaattcaataaagattatataatggaggaaagtcattcctatcttaacacattttgtttatttttaccactagactttgggttattaaggattttattttttatggttttgaggacataacccaggtttttcatacatggtaggcaaatactcttcaattgagttctctctgcagcctgcagatcaaaacaaaacaaaacattatggtaaagcataacaatttacatacttttagttaactgtgaagcattaaataatgatattaagaaaaaaatggaagtaatcctggtagttgatgtgggaggttatatagtgtggtggtttggatatgcttggcctattaggaggtgtggctttgttggagtaggtgtggccttgttggaagaagtacatcattgtgggagtgggctttgacaccctcctcctcgctgcccgaaagacagtattctggctacctttggatcaagatatagaactcttggctccttctccagcaccatgtctgcctgcatgctgttggctaggatgataattgactaaacatctgaaactgtaagccagccccaattaaatgttgtctttctaagaaaaaaaaaaaaaaaa

SEQ ID NO: 2 - protein, 224 aa, Mus musculus
MPHKIEGFFLLLLFGYEATLGLSSTEDEGEDPWYQKACKCDCQVGANALWSAGATSLDCIPECPYHKPLGFESGEVTPDQITCSNPEQYVGWYSSWTANKARLNSQGFGCAWLSKYQDSSQWLQIDLKEIKVISGILTQGRCDIDEWVTKYSVQYRTDERLNWIYYKDQTGNNRVFYGNSDRSSTVQNLLRPPIISRFIRLIPLGWHVRIAIRMELLECASKCA

SEQ ID NO: 3 - DNA, 675 bp, Rattus norvegicus
atgccacacaagattgaaggcttcttcttattgcttctctttggctatgaagccacattgggattgtcttcgacagaggatgagggtgaggacccttggtaccagaaagcgtgcaagtgtgattgccagggaggagccaatgctctgtggtctgctggagccgcctccttagactgtattccagaatgcccatatcacaagcccctgggtttcgagtcaggggaagtcacaccagatcagatcacttgctccaacccagagcagtatgtgggctggtattcctcatggactgcaaacaaggcccggctcaacagtcaaggttttgggtgtgcttggctttccaagtatcaggacagtagccagtggttacagatagatttgaaggagatcaaggtgatttcggggatccttacccaaggacgctgtgacatagatgagtggatgaccaagtacagtgtgcaatataggactgatgaacgcctgaactggatttactataaggatcagactggaaacaatcgggtcttctatggaaactccgaccggagttctacagtccagaacttactgaggccccccattatttcccgcttcatccgactgatccctctaggctggcatgtccgaattgccatccggatggagctgcttgagtgtgccagcaagtgtgcctga

SEQ ID NO: 4 - protein, 224 aa, Rattus norvegicus
MPHKIEGFFLLLLFGYEATLGLSSTEDEGEDPWYQKACKCDCQGGANALWSAGAASLDCIPECPYHKPLGFESGEVTPDQITCSNPEQYVGWYSSWTANKARLNSQGFGCAWLSKYQDSSQWLQIDLKEIKVISGILTQGRCDIDEWMTKYSVQYRTDERLNWIYYKDQTGNNRVFYGNSDRSSTVQNLLRPPIISRFIRLIPLGWHVRIAIRMELLECASKCA

SEQ ID NO: 5 - DNA, 994 bp, Macaca mulatta
cagttcagtaaggtagagcttcggccgaggacgaggggaagatgtcacgcaagatagaaggctttttgctattacttctctttggctatgaagccacattgggattatcgtctaccgaggatgaaggcgaggacccctggtaccaaaaagcatgcaagtgtgattgccaaggaggacccaatgctctgtggtctgcaggtgccacctccttggactgcataccagaatgcccatatcacaagcccctgggtttcgagtcaggggaggtcacaccagaccagatcacctgctctaacccggagcagtatgtgggctggtattcctcgtggactgcaaacaaggcccggctcaacagtcaaggctttgggtgcgcctggctctccaagttccaggacagtagccagtggttacagatagatctgaaggagatcaaggtgatttcagggatccttacccaggggcgctgtgacatcgatgagtggatgaccaagtacagcgtgcagtacaggaccgatgagcgcctgaactggatttactataaggaccagactggaaataaccgggtcttctatggcaactcggaccgcacctccacggttcagaacctgctgcggccccccatcatctcccgcttcattcgcctcatcccgctgggctggcacgtccgcattgccatccggatggagctgctggagtgcgtcagcaagtgtgcctgatgcctgcctcagcttggcgcctgctggggggtgaccggcgcagagcggggccgtaggggaccccctcacataccactgggatggacagggctatatttcgcaaagcaaattttaactgcagtgctgggtagatactttttttttttttttttttaagatatagctttctgatttcaatgaaataaaaatgaacttattccccactcagggccagagaaagtcagaacaaagaaaatgtcccgaaaaccaattttcttacaaaagcctaagcagcaggg

SEQ ID NO: 6 - protein, 224 aa, Macaca mulatta
MSRKIEGFLLLLLFGYEATLGLSSTEDEGEDPWYQKACKCDCQGGPNALWSAGATSLDCIPECPYHKPLGFESGEVTPDQITCSNPEQYVGWYSSWTANKARLNSQGFGCAWLSKFQDSSQWLQIDLKEIKVISGILTQGRCDIDEWMTKYSVQYRTDERLNWIYYKDQTGNNRVFYGNSDRTSTVQNLLRPPIISRFIRLIPLGWHVRIAIRMELLECVSKCA

SEQ ID NO: 7 - DNA, 3039 bp, Homo sapiens
agtaaggtagagctttggccgaggacgaggggaagatgtcacgcaagatagaaggctttttgttattacttctctttggctatgaagccacattgggattatcgtctaccgaggatgaaggcgaggacccctggtaccaaaaagcatgcaagtgcgattgccaaggaggacccaatgctctgtggtctgcaggtgccacctccttggactgtataccagaatgcccatatcacaagcctctgggtttcgagtcaggggaggtcacaccggaccagatcacctgctctaacccggagcagtatgtgggctggtattcttcgtggactgcaaacaaggcccggctcaacagtcaaggctttgggtgtgcctggctctccaagttccaggacagtagccagtggttacagatagatctgaaggagatcaaagtgatttcagggatcctcacccaggggcgctgtgacatcgatgagtggatgaccaagtacagcgtgcagtacaggaccgatgagcgcctgaactggatttactacaaggaccagactggaaacaaccgggtcttctatggcaactcggaccgcacctccacggttcagaacctgctgcggccccccatcatctcccgcttcatccgcctcatcccgctgggctggcacgtccgcattgccatccggatggagctgctggagtgcgtcagcaagtgtgcctgatgcctgcctcagctcggcgcctgccagggggtgactggcacagagcgggccgtaggggaccccctcacacaccaccgagatggacagggctatatttcgcaaagcaattgtaactgcagtgctgggtagataatttttttttttttaagatatagctttctgatttcaatgaaataaaaatgaacttattccccactcagggccagagaaagtcagaacaaagaaaatgtccccgaaacgaattttcttacaaaagcctaagtagcaggggtaattttctgctcattttttgtctcagtgatactgtgaaaggtgcagtctcaggggaacacaaagcagccctgataatttgaaaattcatttgctttaccacattcaagacagaaacatacagtttcctaaagcctggctttgaatgcagaagggagcagctcctcctagttaagtttccactaaatcatcgccaaagaggacttcagagccctggggaggcagctgagggtctcaagggtgactgggtggcagggatgagtgcggtgggtgagaatcccggtgccctgagaggctatacgtgacaaatgaccaaaagcccaaggtaggggagtttcctctgctcacagttcttaccttcaaggcggatctgggcttccaccctcatgaacacagggattggggagggaccagagcgcccaatacacacagctccattatgcaatccattccagcaaattccccgtgtctgtggtcaccatttaggtgatcatacaggacaggctgcacatctcagtatatgtagggaccccaaatgaccacaacacagtacaattgccctttacctagggctaccatttcctagcaaaccaaacatagttcgagaacagctggcccaggagctaccactggctactcagaggaggctcattagctggctacatgcttcgcaggaagtgggaaggactcacatcataaaaaggaccatgtagctttttccctgaaagcttctcaccctccaccctctgccttgcaatacgcaaactgcgcctgctcctgaaaagctctctgggaaggaatgggcctggctttccgttcctggaggcggcgccttagattgggaggcctcattggccacttagagcgcagcctgagtttccaggccccttcctgggagaggctgttaacacgggggaggggcaggagagggatatggagagcaggtggtggaatcagaggacgaggctgctctaaagactgttctggccccagacacagggtagtctttgctagcagctcatttccgagttacttttcattttcaaatgccaaggcaagtgactagactcgcgctaatacagtgctggacaacacattcaccttttctgtgaacaggcagccttctaaaagccccaaacatccttcttgatgctttgggggctcaattattttatatccaacccagcatctttctagtccctatgctgtatgcttgaactcggaaaatgcttttccccgcccaatcttctctcaaatataaacacatcacacagggtgttgggggtggggggggggggtggggggacttatccctggccttaggacacaggacaaatctattttggatagaaatgcctgaacagagacccttatttggaaaggtgaattaactttggtcacgacatggactgtcagacaaaatggcagtatcctaagagttaaggcacatcaaacacaggagtcgagagagtgcagttcagggaaaaaggagaggaggaaacagtgaggcagggagaaaggctttccaaataagagttcatgttggaaacttttgtcacggctttattgagattaagttcacatacaatttgtatccatttaaagtgtacaatttgatgacttttggtatattcagagttgtgcaaccattatcactagatcaattttagaaagtttatcaccccaaagagaaatcctgcacccatcagccaacactccccaacccatcggccaccccaagccctctgcaaccacgaatcgactgtctctgtagattggccttctggacgttctacataaatgaaatcatatagtatgtggtatttcgtgactggcttctttcacttagcatagtgttttaaagttcatccacgttataacatgtgtatcactatgtcacttgtcactcctttttattgctgaacatcattgttcagtatcatgtcaagagcacattgttatttatccattcatccattgatggatatttgggtttccactctttagctattatgaataatgctgctatgaacatttgtgtataaaaaaaaaaaaaaaa

SEQ ID NO: 8 - protein, 224 aa, Homo sapiens; identical to SEQ ID NO: 6

SEQ ID NO: 9 - DNA, 2061 bp, Canis lupus
aatgaggccagcgctcaagttaagcccctgctcctggagaagctctccacttggataaggtagagctgcggccaaggacaaggggagaatgccccgcaagatagaaggcttcttgtttttacttctcttcggctatgaagccacactgggattatcgtctactgaggatgagagtgaggacccctggtaccagaaagcatgcaaatgtgactgccaaggcagtcccaatggcctctggtcggctggtgccacctccttagattgcataccagaatgcccgtatcataagcccctgggtttcgagtcaggagaggttacaccagaccagatcacttgctccaacctggatcagtatgtgggctggtattcctcatggacagctaacaaggcccggctcaacagtcaaggctttgggtgcgcctggctctccaagtaccaggacagcagccagtggttacagatcgatctgaaggaggtcaaggtgatttcaggaatcctcacccaggggcgctgtgacatcgacgagtggatgaccaagtacagcgtgcagtacaggacggatgagaacctgaactggatttactataaggaccagacaggaaacaatcgggtcttctatggaaattcagaccgaacctccacagtccagaaccttctgcggccccccatcatttcccgcttcattcggctgatcccgctgggctggcatgtccgcattgccatccggatggagctgctggaatgcgtcagcaagtgtgcctgaggcctccttcagctccacacctgccctggggtgggggtggggggtagataggggtggagggctcagagcagcctgcaggggaaccctgacagggttccaacagggtgacaaacgcagctgtattttacaagctcttttcaatgcagagcctggcagaaataatttctttaaaaaaacaagtttcccatttcaatcaaagagaaaggaaaacgagcgtatttcccactcactgccaaagaaaataagaacaaagaaaacgtccctaaaactagttttcatctaaaagcctaagtagcaggggtaattttgctgctttttctttttggttttggtctgacagtgtgaaaggtgtggtcccagggaacacaaaagagcccagataatttaaaaactcttttgctttaccacactaaaaacaggaacatagaggtttttcttttcttttcttttcttttcttttcttttcttttcttttcttttcttttcttttcttttcttttctttccggaacacagagtttcataaaaccttgatttgattgcaaatggggagcaagcttgcggtttctccttttaagttttcagtgaatcatggccttttaggacttttagagcacccggcatgcagggggcaaggttttgggtgactggttgtcagagatgagtagagcagttgggagcctgtgtcctggtgtcctgagagctgtgcacaaccaatccccccaggtaagagggcttcctctgctctgagctttcacccccacgcacacaaggatagggagggggtggttgcagagctctcattacatacagatctattctagcaaatttttccagcctgtggtcactatctgggtgaatacatgggacaggctgcacatgtaagcagcagttctctatatttaggaaagccaaatgaccagagctcaccagaatttccccttatctagggctaccatttttcaacaagcttaacattttaaaaacagctggcccaggagctatcactggctacacagaggaagcccattagctaactgcatgctttgcaggaagtggtcagaccctatgtcctaagaagggccatgtggctgtgtctctcacgacccaactgtttaacctctcccccttgccctagaacacacaaccatgcctactcctgaggctgaaatggccttgggagggacggggctaggaatgggcctggccttccgaggggagtgcataaagcagggacttttcagggaccacagcctaagcctcctctgtcatttatagctcagcctgagttttcaggct

SEQ ID NO: 10 - protein, 224 aa, Canis lupus
MPRKIEGFLFLLLFGYEATLGLSSTEDESEDPWYQKACKCDCQGSPNGLWSAGATSLDCIPECPYHKPLGFESGEVTPDQITCSNLDQYVGWYSSWTANKARLNSQGFGCAWLSKYQDSSQWLQIDLKEVKVISGILTQGRCDIDEWMTKYSVQYRTDENLNWIYYKDQTGNNRVFYGNSDRTSTVQNLLRPPIISRFIRLIPLGWHVRIAIRMELLECVSKCA

SEQ ID NO: 11 - DNA, 1772 bp, Sus scrofa
ccgggtcttctgattccagtttctattttcctccactgcttcccttacatttaaagatagaataaagccagtagcttcctttgctaaaccgacctcagttgacatcggcttcttctcagagacttccttgttgaggcaggtaacgacgtgggttaacttgtcggggctcagccaaagccctaagagctaaatggaataagatgcttaatgaggccagtgctcaagttaagctcctgttcctagggaagctctccacttcgataaggaagagcagcagccaaggacaaggggagaatgccacgcaagatagaaggcttcttgtttttacttctctttggctatgaagccaccctgggattatcgtctacggaggatgagggtgaggacccctggtacaacaaagcgtgcaagtgtgactgccaaggaggcgccaatgccctgtggtctgcgggcaccacccccttagactgcataccggaatgcccgtatcataagcccctggggttcgagtcaggagaggttacaccagaccagattacctgctccaacctggagcagtacgtgggctggtattcctcgtggactgccaacaaggcccggctcaacagtcaaggctttgggtgcgcctggctctccaagttccaggacagcagccagtggttacagatagatctgaaggaggtcaaggtgatttcagggatcctcacccagggccgctgtgacatcgatgagtggatgaccaagtacagcgtgcagtacaggaccgatgagagcctgaactggatttactataaggaccagactggaaacaaccgggttttctatggaaactcagaccgaacctccacagtccagaacctgctacggccccccatcatttcccgcttcatccggctcatcccgctgggctggcacgtgcgcattgccatccggatggagttgctggagtgcgtcagcaagtgtacctgacggggtgcccgccagggtgcgcagggcacggagcagccgggcgactgctgatctaccgctgtgaccaacaaggctgtatcttacaggctctactcaatgcagagctgggcagagaagacatctttctttctttggttttcttcctttctttttttttaaatatagtttgcatttcaataaacaaaccgaattaaatcttcactcagggccaaagaaaataagaacaaagaaaatgtccctaaaaacaattttcatgcaaaagcaaagcaggagtaatttgctgctctctggagttttttgttttcgcttttttttttttttttttttttgattgtttgctttttggtctcagtgacactgtgcaaggtgccctcccaggagaatgcaaagcagccctaataatctgaaaattcttttgctttaccacattcaaaacaagaacacagagtttcataaagcctcactttgaaagcaaagagggagcaagcttgtgggttctcctagcttcgttttcattaaatcatggccttttagaacttgagagcactgggtatgcagggtaaaaggttctggagtgactaggagggtgggagcccattttacggtcccctgagagccaggtaggagggcctcccctgctcagagtttcacccccagtcagtgcaatttatcctagtctgtggtcactacttaggtgaataatggacaggctgcacatgtatgtagccaagtctccctatatttaggaacctcaaatgaccagaacacaccagaatttccttttatctagggtaaccatttaa

SEQ ID NO: 12 - protein, 224 aa, Sus scrofa
MPRKIEGFLFLLLFGYEATLGLSSTEDEGEDPWYNKACKCDCQGGANALWSAGTTPLDCIPECPYHKPLGFESGEVTPDQITCSNLEQYVGWYSSWTANKARLNSQGFGCAWLSKFQDSSQWLQIDLKEVKVISGILTQGRCDIDEWMTKYSVQYRTDESLNWIYYKDQTGNNRVFYGNSDRTSTVQNLLRPPIISRFIRLIPLGWHVRIAIRMELLECVSKCT

SEQ ID NO: 13 - DNA, 899 bp, Bos taurus
ctccactttgataaggaagagcagcagccaaggacaaggggagaatgccacgcaagatagaaaacttcttgtttttacttctcttcggctatgaagccacactgggattatcatctactgaggatgagggtgaagatccctggtaccacaaagcgtgcaagtgcgattgccaaggaggtgccaatgccctgtggtctgcaggtcccacccccttggactgcataccggaatgcccataccataagcccctgggtttcgagtcaggagaggttacaccagaccagatcacctgctccaacgtggagcagtacgtgggctggtattcttcctggactgccaacaaggcccggcttaacagtcaaggctttgggtgtgcctggctctccaagttccaggacagcagccagtggttacagatagatctgaaggaggtcaaggtgatttcggggatcctcacccaggggcgctgtgacatcgatgagtggatgaccaagtacagtgtgcagtacaggaccgatgagagtctgaactggatttactataaagaccagaccggaaacaaccgggttttctatggaaattcggaccgaacctccacagtccagaacctgctgcggccccccatcatctcccgcttcatccggctcataccgctaggctggcatgttcgcattgccatccggatggagctgctggagtgcgtcagcaagtgtacctgatgttgcctcggctcatacctgcagtgggtgaagggtgcagagcggcccatgggggaacgctgacttatcactgtgaccagcagggctggattttacaggctcttttcagcgcagggctgggcagagaatactatcttttttgcatagtttccaatttcagtgagagaaaatgaaaatgaa

SEQ ID NO: 14 - protein, 224 aa, Bos taurus
MPRKIENFLFLLLFGYEATLGLSSTEDEGEDPWYHKACKCDCQGGANALWSAGPTPLDCIPECPYHKPLGFESGEVTPDQITCSNVEQYVGWYSSWTANKARLNSQGFGCAWLSKFQDSSQWLQIDLKEVKVISGILTQGRCDIDEWMTKYSVQYRTDESLNWIYYKDQTGNNRVFYGNSDRTSTVQNLLRPPIISRFIRLIPLGWHVRIAIRMELLECVSKCT

SEQ ID NO: 15 - DNA, 1604 bp, Ovis aries
actttgacttcttccagaaggggccttgttaactttttatgtgactattatcactttgcttttccgtgtaatgagtcatttgttgaatttttctttcttgttttaacttgatttttcctctcttgtccttttgctcagccacactgggattatcatctactgaggtatgttacagtaagaaggctggaattcatacggatactgtttttgaacattttcatagccaaaaacaatgtataggattatcacttctttaaaaatgtatttttaaacatatattttttctggtggtggaaatagcatgttttatctggacaaagttcaagactgattcagataaatgagacaatgcaagtgaaccaggtcttatgtcagatggcagaatcttgaattcagtcccttttaaaactggatccccagaagggccctgcagatgtgaggagcctgactggaagatcactacaatggggtggacacggctctctacataggtgtgtctgtgaagtttttagctggtcatccacagtgacaaacatttgtctatttagactcaaagatgagtggtgactgtgtgttaaactgggttcataagtcagttgcactgctgtagagtgaaagctgccctagacaataggaactaaatgagtgaggtttgtgaatgcaagcttttccagtagttctgaccacagttgcctttgactatggcttttctgaagttcctgccccctgatttcccgcaggatgagggtgaggatccctggtaccacaaagcatgcaagtgtgattgccaaggaggtgccaatgccctgtggtctgcaggttccacccccttggactgcataccggaatgcccataccataagcccctgggtttcgagtcaggagaggttacaccagaccagatcacctgctccaacgtggagcagtacgtgggctggtattcttcctggactgccaacaaggcccggctcaacagtcaaggctttgggtgcgcttggctctccaagttccaggacagcagccagtggttacagatagatctgaaggaggtcaaggtgatttcggggatcctcacccaggggcgctgtgacatcgatgagtggatgaccaagtacagtgtgcagtacaggaccgatgagagcctgaactggatttactataaagaccagactggaaacaaccgggttttctatggaaattcggaccgaacctccacagtccagaacctgctgcggccccccatcatctcccgcttcatccggctcatcccactaggctggcatgtccgcattgccatccggatggagctgctggagtgcgtcagcaagtgtacctgatgctgcctcggctcatgcctgcagtgggtgaagggcgcagagtggcccatgggggaactctgacttatcactgtgaccaacagggctggattttacaggctcttttcagtgcagggctgggcagagaatactatcttttttgcatagtttccaatttcagtaagagaaaatgaaaataaacgtatttcccattcagggtcaaagaaaataagaacaaagaaaatgtctctaaaaacaatttccatgcagaaagcctaagtagcagga

SEQ ID NO: 16 - protein, 211 aa, Ovis aries
MAFLKFLPPDFPQDEGEDPWYHKACKCDCQGGANALWSAGSTPLDCIPECPYHKPLGFESGEVTPDQITCSNVEQYVGWYSSWTANKARLNSQGFGCAWLSKFQDSSQWLQIDLKEVKVISGILTQGRCDIDEWMTKYSVQYRTDESLNWIYYKDQTGNNRVFYGNSDRTSTVQNLLRPPIISRFIRLIPLGWHVRIAIRMELLECVSKCT

SEQ ID NO: 17 - DNA, 4553 bp, Felis catus
cttctgaggaaaccctccactcggataaggtagagctacagccaaggacaaggggagaatgccacgcaagatagaaggtttcttgttcttacttctctttggctacgaagccacactgggactgtcgtctactgaggatgagggtgaggacccctggtaccacaaagcatgcaaatgcgattgccaaggaggtgccaatgccctctggtctgctggcgccacctccttagactgcattccggaatgcccatatcataagcccctgggtttcgaatcgggagaagttacaccagaccagatcacctgctccaacctggagcagtacgtgggctggtattcctcgtggaccgctaacaaggcccggctcaacagtcaaggctttgggtgcgcctggctgtccaagtaccaggacagcagccagtggctagagatagatctgaaggaggtcaaggtgatttcagggatcctcacccaggggcgctgtgacattgatgagtggatgaccaagtacagcgtgcagtacaggaccgatgagaacctgaactggatttactataaggaccagacaggaaacaaccgggtcttctacggcaactcagaccgaacctccacggtccagaacctcctgcggccccccatcatttcccgcttcatccggctgatcccactgggctggcacgtccgcattgccatccggatggagctgttggagtgcgtcagcaagtgtgcgtgacgcctccttcagctcggcacctgccaggtggggtggagggcgcagagcagcctgtaggggaaaattgacgcgaccagggcttgaacagggtgacaaacagggctgaattttacaagctcttttcaatgcagagctgggcagaaataatttcttttttttaagacgtagtttccaatgtcaatgagagagaaagaaaaatgaactcattccccactcagggccaaagaaaataagaacaaagaaaatgtccctaaagacaatgttcatcaaaagcctaagtagcaggggtaattttctgctcttgggtttttgtgtttggcctgacagtgtgaaaggtgtggtctcagggaacacaaaggagcccagataatttaaaaacccttttgcttcaccaccctgaaaacaggaacagaagtttcataaaaccttgatttgaacgcaaatgggtagcaggcttgcggtctctccggcgttttcaccaaattagggcctctcacaactttagagcaccgtgtatgcagacggaaaggatttggggtgactggggggccgaaaggcatagtcgggagcctgtgtcctggtctcctggaggctggcaccatcaccccaggcaggagggcctcccctgctctgcgccttcacccccacgcacacaaggactgtggagccacaaaagctctcatcacatacagatccattctagcaaagttttccagtctgtggtcactatttgggtaaatacatgggacgggctgcatgtgtaagtagcaaagtttctctgtatttaggaaccccacatgaccgaagcacaccagaatttcccttcatctagggctaccatttttcaacaggattcacattttaaaaccagttggcacaggagctagatcactggctacacggaggaggcccatcagctaaccacatgctttgcaggaagtgggcagaccgcaagtcctaagaagggatgtggatacgtttcttgtgacccacggttaaacttcaccccttgccttgcaacacacaaaacaggcctgctcctgaggttgaaacctccttgagaaggaccgggcctggcatgggcctggccttccccctcctggaggagctcatgaagctgggacctttcgggaagagtctcagtctcctgagttttcaggcccttccctggggagaggctgatgacatggggagtgggcaggagaggtatatgaaagtaggagctgagagggggtgaaactgggggatgagggccctctgacaagactggggaatccgagactgtcctggccctgacacagcacagcctctactagaggctttctcctgagttactttctgttttcaaatgccaagccgagtgaagactcacactaacatgatcctggacatcacattcaccttctctgtgagggggaagcctcctaaaaaccccaaatctcttccctggtgttttgggcttagaacagctctatatttaacccaccatccttttttttttttttttttttttttttaacgtttattttgaaagagagaggagagagagagagggagagagcatgcatacgcacgcgagcaagcagagaagggtcagatagagagggagacagaggatctgaagcgggctctgcacggtcagcagtgagcctgatgtggggccgaacttgtgacctgtgagatcatgacctgagctgaagtcggacgcttaaccgactgagccgcccaggtgcccctaacccaccatctttttaatcccccaactgtatacttggacctggaaaaatgcttcccttgctcagtattctctcaaatacaaacatatcaaattcaaggtggggaaaaaaaaatccttctctggactttggacacatgaataaatccatttagagcaggcgcctcatcagagccccttagtgaaaagctgaatgaactttcatcatgacacggattgtcagagaaaatggtggtagcctaagagctcaggtcctctacagtggtcacatcagacacaggaggcgagtacggttaagaggaaagaagaaaagaatgaaactgtgaggcagtgataaaggttctccaactaattgttcatgttagaaatgtttgctttgtaaaggtttaatgagataaagtcacataccgtacaaatttcaaccatttcaagtgtacaattcaatgacttttagtagactcagagttgaggaaccattatcacaattttagaaaaatttcatcaccccacagagaaaccctgcacccattaaccatcacctcccaacctactcgtccccgcagccctaggcaaccactgatggactttctgtctcagtagatttgcctattctggacatttcatataaatgggatcattttctgcctggcttcttttgcttagcatagtgtttttccaagtttcattcaggttgcagcatgcacttaattccttcttatagctgaacatcattccgttatatggataggtcacattgtatttatccgttcatctgttgatggacatttgggttgtttctacatttttggctatcgtgaataatgctgctataaacacctgtgtacaagtttttgtttggacatatgtttttatttatcttgggcatatacctaggagtggaatgctggggtcatatggtaactctacgtctaacctttttaggaactgtcagacaattttccaaaggggccacaccattatgcattcccaccagcaacatatgagagtttcaggttctctacatttgttattatctttttgattagagccgtcctggtgtgtatgaagtagcatcactctggtttttgatttgcatttccctaggactaatgatgctaagcatcttttttatgtgttcactggccttttgaataacttctttggagaaatgtcttttccgatcctttgcccatttaaaaatcaggtggcctttttattaacgaattgtaagagctctttaatattctagatacaacccccttaggagatacgtgacttgcaaatactttctcctattcggtaggttatcttcttactctcttgatggagtcctttgaaacacatttttaaattttgataaagtccaatttattcttttttgttgcatgtgtttttggtgtcatatctgaggtaccattgccaaatcccgatcatgaagatttactcctatgtttcaagagttttatagttttacttcttacatttagacctttgatctatttggggttattttgtatatggtatgaggtaggggtccaacttcagtatctgcacgtggacatccagttgtcccagcaccatttgttgaaaagactttttccccactgaatggtcttggcatcctttttgagaaatcaattaaccataaaggtgagaatttgtttctggatcctcaattctattccattataggtctatctttataccagtaccacacagttgtcattactgtagcctttttagtaagttttgaaattggaacaggttaactctccaactttgttcttcttcaaggctgtctgggctgctgagtcctttgaatgtccatatgaattttagaatcactgtgtcaatttctgcaaagaagccagctgagatttcacatcggaaatcgctccatacttgagaatttaatcaacaatgagatactgagatccataatacgttaatctgtaggtaacctgtgtataacagcatattaattatttacttcatttaatttagaacagaaagtataaaaacaaaacttttattgaggggcatctgcagcctaacagaatcttgctattaaacacatgaactgtg

SEQ ID NO: 18 - protein, 224 aa, Felis catus
MPRKIEGFLFLLLFGYEATLGLSSTEDEGEDPWYHKACKCDCQGGANALWSAGATSLDCIPECPYHKPLGFESGEVTPDQITCSNLEQYVGWYSSWTANKARLNSQGFGCAWLSKYQDSSQWLEIDLKEVKVISGILTQGRCDIDEWMTKYSVQYRTDENLNWIYYKDQTGNNRVFYGNSDRTSTVQNLLRPPIISRFIRLIPLGWHVRIAIRMELLECVSKCA

SEQ ID NO: 19 - DNA, 1193 bp, Equus caballus
atgccacacaaaatagaaggcttcttgtttttacttctctttggctatgaagccacactgggattatcgtctactgaggatgagggcgaggacccctggtaccacaaagcgtgcaagtgcgattgccaaggaggcaccaacaccctgtggtctgtgggtgccacctccttagactgcataccggaatgcccataccataagcccctgggtttcgagtcaggagaggtgaccccagagcagatcacctgctccaacccggagcagtacgtgggctggtactcctcgtggaccgccaacaaggcccggctcaacagtcaaggctttgggtgcgcctggctctccaaattccaggacagcagccagtggttacagatagacctgaaggaggtcaaggtgatttcagggatcctcacccaggggcgctgtgacatcgacgagtggatgaccaagtacagcgtgcagtacaggactgatgagagcctgaactggatttactataaggaccagaccggaaataaccgggtcttctatggaaactcagaccgaacctccacagtccagaacctgctgcggcccccaattatttcccgcttcatccggctgatcccactgggctggcacgtccgcatcgccatccggatggagctgctggagtgtgtcagcaagtgtccctgacgcctcctgcctcagcctcggccctcggggggagggcgcagagggcctgggggaccctgatgccgcactgtgacaaacaaggccgtattttacaagctgctctcgggttttttttgtctccatgatgctgtgaaaggtgcagtcccaggggaacacgaagcagccctgatcattcgagaattcttgtgctttaccacgttcaaaacaggaacagagagtttcataaaccctcactttgaatgcaaagggggagcaagcttgcagtttctcctagctaggttttcgttaaatcagggcctcttaggactttagagcaccgggtaggcagagtgaaagttttggggctgactgggtggcggcgttgagtatggtggatgggagcctgtgtcctggtctcctgagagccatacacgtccaaacgcctcacgtaggatggcctcccctgccccgggctctcgtctcctgcacacagagattgtgcatgggcccatgctgcagcccatttcaggccaactgtc

SEQ ID NO: 20 - protein, 224 aa, Equus caballus
MPHKIEGFLFLLLFGYEATLGLSSTEDEGEDPWYHKACKCDCQGGTNTLWSVGATSLDCIPECPYHKPLGFESGEVTPEQITCSNPEQYVGWYSSWTANKARLNSQGFGCAWLSKFQDSSQWLQIDLKEVKVISGILTQGRCDIDEWMTKYSVQYRTDESLNWIYYKDQTGNNRVFYGNSDRTSTVQNLLRPPIISRFIRLIPLGWHVRIAIRMELLECVSKCP

SEQ ID NO: 21 - DNA, 675 bp, Oryctolagus cuniculus
atgctacgcaagatggaaggcttcttgttcttacttctctttggctatgaagccacactgggattatcgtctactgaggatgagagtgaggacccgtggtaccacaaagcgtgcaagtgcgactgccaaggaggagccaatgccctgtggaatgcaggtgccacctccttagactgcataccagaatgcccgtatcacaagcccctgggtttcgagtcaggggaagtgacagcagaccagatcacctgctccaatccggagcagtatgtgggctggtattcctcgtggaccgcaaacaaggcccggctcaatagtcaaggctttgggtgcgcttggctctccaagttccaggacagcagccagtggttacagatagacctgaaggagatcaaggtgatttcgggcatcctcacccaaggacgctgtgacatcgatgagtggatgaccaagtacagtgtgcagtacaggaccgatgagcgcctgaactggatttactacaaggaccagaccggaaacaaccgggtcttctatggcaactcggaccgaagctccacagtccagaacctgctgcggccaccgatcatctcccgcttcatccggctgatcccgctgggctggcacgtccgcattgccatccggatggagctgctggagtgtgtcagcaagtgtgcctga

SEQ ID NO: 22 - protein, 224 aa, Oryctolagus cuniculus
MLRKMEGFLFLLLFGYEATLGLSSTEDESEDPWYHKACKCDCQGGANALWNAGATSLDCIPECPYHKPLGFESGEVTADQITCSNPEQYVGWYSSWTANKARLNSQGFGCAWLSKFQDSSQWLQIDLKEIKVISGILTQGRCDIDEWMTKYSVQYRTDERLNWIYYKDQTGNNRVFYGNSDRSSTVQNLLRPPIISRFIRLIPLGWHVRIAIRMELLECVSKCA

SEQ ID NO: 23 - DNA, 8202 bp, Artificial Sequence
  recombinant or synthetic polynucleotide
ggtaccgatttaaatgatccagtggtcctgcagaggagagattgggagaatcccggtgtgacacagctgaacagactagccgcccaccctccctttgcttcttggagaaacagtgaggaagctaggacagacagaccaagccagcaactcagatctttgaacggggagtggagatttgcctggtttccggcaccagaagcggtgccggaaagctggctggagtgcgatcttcctgaggccgatactgtcgtcgtcccctcaaactggcagatgcacggttacgatgcgcccatctacaccaacgtgacctatcccattacggtcaatccgccgtttgttcccacggagaatccgacgggttgttactcgctcacatttaatgttgatgaaagctggctacaggaaggccagacgcgaattatttttgatggcgttaactcggcgtttcatctgtggtgcaacgggcgctgggtcggttacggccaggacagtcgtttgccgtctgaatttgacctgagcgcatttttacgcgccggagaaaaccgcctcgcggtgatggtgctgcgctggagtgacggcagttatctggaagatcaggatatgtggcggatgagcggcattttccgtgacgtctcgttgctgcataaaccgactacacaaatcagcgatttccatgttgccactcgctttaatgatgatttcagccgcgctgtactggaggctgaagttcagatgtgcggcgagttgcgtgactacctacgggtaacagtttctttatggcagggtgaaacgcaggtcgccagcggcaccgcgcctttcggcggtgaaattatcgatgagcgtggtggttatgccgatcgcgtcacactacgtctgaacgtcgaaaacccgaaactgtggagcgccgaaatcccgaatctctatcgtgcggtggttgaactgcacaccgccgacggcacgctgattgaagcagaagcctgcgatgtcggtttccgcgaggtgcggattgaaaatggtctgctgctgctgaacggcaagccgttgctgattcgaggcgttaaccgtcacgagcatcatcctctgcatggtcaggtcatggatgagcagacgatggtgcaggatatcctgctgatgaagcagaacaactttaacgccgtgcgctgttcgcattatccgaaccatccgctgtggtacacgctgtgcgaccgctacggcctgtatgtggtggatgaagccaatattgaaacccacggcatggtgccaatgaatcgtctgaccgatgatccgcgctggctaccggcgatgagcgaacgcgtaacgcgaatggtgcagcgcgatcgtaatcacccgagtgtgatcatctggtcgctggggaatgaatcaggccacggcgctaatcacgacgcgctgtatcgctggatcaaatctgtcgatccttcccgcccggtgcagtatgaaggcggcggagccgacaccacggccaccgatattatttgcccgatgtacgcgcgcgtggatgaagaccagcccttcccggctgtgccgaaatggtccatcaaaaaatggctttcgctacctggagagacgcgcccgctgatcctttgcgaatacgcccacgcgatgggtaacagtcttggcggtttcgctaaatactggcaggcgtttcgtcagtatccccgtttacagggcggcttcgtctgggactgggtggatcagtcgctgattaaatatgatgaaaacggcaacccgtggtcggcttacggcggtgattttggcgatacgccgaacgatcgccagttctgtatgaacggtctggtctttgccgaccgcacgccgcatccagcgctgacggaagcaaaacaccagcagcagtttttccagttccgtttatccgggcaaaccatcgaagtgaccagcgaatacctgttccgtcatagcgataacgagctcctgcactggatggtggcgctggatggtaagccgctggcaagcggtgaagtgcctctggatgtcgctccacaaggtaaacagttgattgaactgcctgaactaccgcagccggagagcgccgggcaactctggctcacagtacgcgtagtgcaaccgaacgcgaccgcatggtcagaagccgggcacatcagcgcctggcagcagtggcgtctggcggaaaacctcagtgtgacgctccccgccgcgtcccacgccatcccgcatctgaccaccagcgaaatggatttttgcatcgagctgggtaataagcgttggcaatttaaccgccagtcaggctttctttcacagatgtggattggcgataaaaaacaactgctgacgccgctgcgcgatcagttcacccgtgcaccgctggataacgacattggcgtaagtgaagcgacccgcattgaccctaacgcctgggtcgaacgctggaaggcggcgggccattaccaggccgaagcagcgttgttgcagtgcacggcagatacacttgctgatgcggtgctgattacgaccgctcacgcgtggcagcatcaggggaaaaccttatttatcagccggaaaacctaccggattgatggtagtggtcaaatggcgattaccgttgatgttgaagtggcgagcgatacaccgcatccggcgcggattggcctgaactgccagctggcgcaggtagcagagcgggtaaactggctcggattagggccgcaagaaaactatcccgaccgccttactgccgcctgttttgaccgctgggatctgccattgtcagacatgtataccccgtacgtcttcccgagcgaaaacggtctgcgctgcgggacgcgcgaattgaattatggcccacaccagtggcgcggcgacttccagttcaacatcagccgctacagtcaacagcaactgatggaaaccagccatcgccatctgctgcacgcggaagaaggcacatggctgaatatcgacggtttccatatggggattggtggcgacgactcctggagcccgtcagtatcggcggaattccagctgagcgccggtcgctaccattaccagttggtctggtgtcaaaaataataataaccgggcaggggggatctaagctctagataagtaatgatcataatcagccatatcacatctgtagaggttttacttgctttaaaaaacctcccacacctccccctgaacctgaaacataaaatgaatgcaattgttgttgttaacttgtttattgcagcttataatggttacaaataaagcaatagcatcacaaatttcacaaataaagcatttttttcactgcattctagttgtggtttgtccaaactcatcaatgtatcttatcatgtctggatcccccggctagagtttaaacactagaactagtggatccccgggctcgataactataacggtcctaaggtagcgactcgacataacttcgtataatgtatgctatacgaagttatatgcatgccagtagcagcacccacgtccaccttctgtctagtaatgtccaacacctccctcagtccaaacactgctctgcatccatgtggctcccatttatacctgaagcacttgatggggcctcaatgttttactagagcccacccccctgcaactctgagaccctctggatttgtctgtcagtgcctcactggggcgttggataatttcttaaaaggtcaagttccctcagcagcattctctgagcagtctgaagatgtgtgcttttcacagttcaaatccatgtggctgtttcacccacctgcctggccttgggttatctatcaggacctagcctagaagcaggtgtgtggcacttaacacctaagctgagtgactaactgaacactcaagtggatgccatctttgtcacttcttgactgtgacacaagcaactcctgatgccaaagccctgcccacccctctcatgcccatatttggacatggtacaggtcctcactggccatggtctgtgaggtcctggtcctctttgacttcataattcctaggggccactagtatctataagaggaagagggtgctggctcccaggccacagcccacaaaattccacctgctcacaggttggctggctcgacccaggtggtgtcccctgctctgagccagctcccggccaagccagcaccatgggaacccccaagaagaagaggaaggtgcgtaccgatttaaattccaatttactgaccgtacaccaaaatttgcctgcattaccggtcgatgcaacgagtgatgaggttcgcaagaacctgatggacatgttcagggatcgccaggcgttttctgagcatacctggaaaatgcttctgtccgtttgccggtcgtgggcggcatggtgcaagttgaataaccggaaatggtttcccgcagaacctgaagatgttcgcgattatcttctatatcttcaggcgcgcggtctggcagtaaaaactatccagcaacatttgggccagctaaacatgcttcatcgtcggtccgggctgccacgaccaagtgacagcaatgctgtttcactggttatgcggcggatccgaaaagaaaacgttgatgccggtgaacgtgcaaaacaggtaaatataaaatttttaagtgtataatgatgttaaactactgattctaattgtttgtgtattttaggctctagcgttcgaacgcactgatttcgaccaggttcgttcactcatggaaaatagcgatcgctgccaggatatacgtaatctggcatttctggggattgcttataacaccctgttacgtatagccgaaattgccaggatcagggttaaagatatctcacgtactgacggtgggagaatgttaatccatattggcagaacgaaaacgctggttagcaccgcaggtgtagagaaggcacttagcctgggggtaactaaactggtcgagcgatggatttccgtctctggtgtagctgatgatccgaataactacctgttttgccgggtcagaaaaaatggtgttgccgcgccatctgccaccagccagctatcaactcgcgccctggaagggatttttgaagcaactcatcgattgatttacggcgctaaggatgactctggtcagagatacctggcctggtctggacacagtgcccgtgtcggagccgcgcgagatatggcccgcgctggagtttcaataccggagatcatgcaagctggtggctggaccaatgtaaatattgtcatgaactatatccgtaacctggatagtgaaacaggggcaatggtgcgcctgctggaagatggcgattaggcggccggccgctaatcagccataccacatttgtagaggttttacttgctttaaaaaacctcccacacctccccctgaacctgaaacataaaatgaatgcaattgttgttgttaacttgtttattgcagcttataatggttacaaataaagcaatagcatcacaaatttcacaaataaagcatttttttcactgcattctagttgtggtttgtccaaactcatcaatgtatcttatcatgtctggatcccccggctagagtttaaacactagaactagtggatcccccgggatcatggcctccgcgccgggttttggcgcctcccgcgggcgcccccctcctcacggcgagcgctgccacgtcagacgaagggcgcagcgagcgtcctgatccttccgcccggacgctcaggacagcggcccgctgctcataagactcggccttagaaccccagtatcagcagaaggacattttaggacgggacttgggtgactctagggcactggttttctttccagagagcggaacaggcgaggaaaagtagtcccttctcggcgattctgcggagggatctccgtggggcggtgaacgccgatgattatataaggacgcgccgggtgtggcacagctagttccgtcgcagccgggatttgggtcgcggttcttgtttgtggatcgctgtgatcgtcacttggtgagtagcgggctgctgggctggccggggctttcgtggccgccgggccgctcggtgggacggaagcgtgtggagagaccgccaagggctgtagtctgggtccgcgagcaaggttgccctgaactgggggttggggggagcgcagcaaaatggcggctgttcccgagtcttgaatggaagacgcttgtgaggcgggctgtgaggtcgttgaaacaaggtggggggcatggtgggcggcaagaacccaaggtcttgaggccttcgctaatgcgggaaagctcttattcgggtgagatgggctggggcaccatctggggaccctgacgtgaagtttgtcactgactggagaactcggtttgtcgtctgttgcgggggcggcagttatggcggtgccgttgggcagtgcacccgtacctttgggagcgcgcgccctcgtcgtgtcgtgacgtcacccgttctgttggcttataatgcagggtggggccacctgccggtaggtgtgcggtaggcttttctccgtcgcaggacgcagggttcgggcctagggtaggctctcctgaatcgacaggcgccggacctctggtgaggggagggataagtgaggcgtcagtttctttggtcggttttatgtacctatcttcttaagtagctgaagctccggttttgaactatgcgctcggggttggcgagtgtgttttgtgaagttttttaggcaccttttgaaatgtaatcatttgggtcaatatgtaattttcagtgttagactagtaaattgtccgctaaattctggccgtttttggcttttttgttagacgtgttgacaattaatcatcggcatagtatatcggcatagtataatacgacaaggtgaggaactaaaccatgggatcggccattgaacaagatggattgcacgcaggttctccggccgcttgggtggagaggctattcggctatgactgggcacaacagacaatcggctgctctgatgccgccgtgttccggctgtcagcgcaggggcgcccggttctttttgtcaagaccgacctgtccggtgccctgaatgaactgcaggacgaggcagcgcggctatcgtggctggccacgacgggcgttccttgcgcagctgtgctcgacgttgtcactgaagcgggaagggactggctgctattgggcgaagtgccggggcaggatctcctgtcatctcaccttgctcctgccgagaaagtatccatcatggctgatgcaatgcggcggctgcatacgcttgatccggctacctgcccattcgaccaccaagcgaaacatcgcatcgagcgagcacgtactcggatggaagccggtcttgtcgatcaggatgatctggacgaagagcatcaggggctcgcgccagccgaactgttcgccaggctcaaggcgcgcatgcccgacggcgatgatctcgtcgtgacccatggcgatgcctgcttgccgaatatcatggtggaaaatggccgcttttctggattcatcgactgtggccggctgggtgtggcggaccgctatcaggacatagcgttggctacccgtgatattgctgaagagcttggcggcgaatgggctgaccgcttcctcgtgctttacggtatcgccgctcccgattcgcagcgcatcgccttctatcgccttcttgacgagttcttctgaggggatccgctgtaagtctgcagaaattgatgatctattaaacaataaagatgtccactaaaatggaagtttttcctgtcatactttgttaagaagggtgagaacagagtacctacattttgaatggaaggattggagctacgggggtgggggtggggtgggattagataaatgcctgctctttactgaaggctctttactattgctttatgataatgtttcatagttggatatcataatttaaacaagcaaaaccaaattaagggccagctcattcctcccactcatgatctatagatctatagatctctcgtgggatcattgtttttctcttgattcccactttgtggttctaagtactgtggtttccaaatgtgtcagtttcatagcctgaagaacgagatcagcagcctctgttccacatacacttcattctcagtattgttttgccaagttctaattccatcagacctcgacctgcagcccctagataacttcgtataatgtatgctatacgaagttatgctagc

SEQ ID NO: 24 - DNA, 13716 bp, Artificial Sequence
  recombinant or synthetic polynucleotide
ccacacaagattgaaggcttcttcttgttacttctctttggctatgaaggtatgtactattctactattggcatttattaatgtatttaataatgtgatttaatatagaaatatatagaaaatagttgataaatagaaatgcaacctgagtaataaaaattgttggatgacaacatgccaattagttcacaggttattaatttaaaaggtcactgttgtgtggctctttgtcactgtcttgctcctggcttcctggtttcatgaggaaccttctaaagttcaaatgatattgaaactcaacagaaagaaggaagggcctcagagtttctataaaaacaactttaaattgcaacaattaatgagaagtcatgtttcttggaaattttaggaggcaaagttgaagcaattgtagaatttaatattgtaagccggactattactgagggttaaggatgaagctattaatagctctgctgggacaagtgtaaatgaggactgtcccaggcaaatcaggacaaagggtcaccctagtttaaatatggattagcataaggccaagcaccactgcagtctaatagaagtctaataaaataatccaaagaaagtcaataaaccctaaagactcaatatattccatcacttttaaacttctaaatgtggccctggcaggcataatatgcttaaataaggacagattaaagctaaatctctaaaatgtcaatcaaataaactttaaatctctttccatcttagacataatactctctcatgcctctcttacctctctagtgcccatcaattcagaattccttttaaagtttatactttcaaatattaaaaattggttgaagggttggggatgtggctcagtggtacagcccctgcccagccttcatgagtccctgagttaaattcccagaagcagtataagacaaacaaacaaaaaccttacttcatccattttctggcatagctacacatacctgcaatcctagttctggacaaattcaagcaggagcattcaatgccaacctcagctacttaggtttgggctatctgagaccctgtcttaacattgggggagagcctaggctaggctgagctatacagtaagcctctgtctgggaaggagggaaaaaggaaggaaagacattggttgaatgacttgtgggtgacactgtatgtttagagtgttcagggaaaaggaggcctctctgctctgcaaatgacctgccactcagataagacgaatacacacaagagtcagaattcctctgtttcttctatattcatgaaccagcagtcttgtgtcttttattatctaataatatttctagtgtctggaaagccttgtgaaaataaaatctcaaggtcatacggcaaacacaaagaaacaggtttttttttcttttttttctttttttttttttatacatatttgttttatttatttatttattatatgtacgtacactgtagctgtcttcagacactccagaagagggcatcagatctcgttacggatggttgtgagccaccatgtggttgctgggatttgaacttcagaccttcggaagagcagtcgggtgctcttacccactgagccatctcaccagccccaggttttttttttcttagttgttattattattgttattcttttgagacaggatcccacactgaaactcaggctagccttcaatttcctatggatttgacctcatagcagtcagccagtttccaccttctgagtgctaagatttcaagcctgagccaccacacccaattcctaagatatgtttttaagcaaggttattggcattacaccttaaccctttgcaatgacgtgtcaggaatttgcaccttttttttttttccagttgtcaggcctggcaatggagcccagggccctgtgcttgctaaacgatggctctacccctaagttatatatacccagcttatcccaggatctttctcagactttctgatgtttgctatcgatgttgcttctctttggttccttgctcttttctcacaaaaagatctaagcaagaacccttgtctggagtcagagagatagcttagtctggaaagtgcttatagcttacacacagaaacttgagttcgatccccagaacttttcttgtttaaaaaacaaacaaacaaacaaacaaaaactaggcatgacagctggagaggtggcttcgcaattaacagcacttgttaaagaggacctcagcttggttcccagggctctataactccagttccagggcctcagacagcctcctgtagcctcttcatgcatcagacatggtccatatgcatgcaggtcaaacactcatacacattaaatgaaaaataaaagtctaaaaaaaggtcaaacatagtgatgcatgctataatcccagtgctagggaggcaaatgtctggaccttgtcggtcggccagtcagtcagccagccagtcagtctagcctagcatagcctactaggtgtgctccagcccaatgagagaccttgtctctaaaaaaaagggtagaaagaaaagacaaaatggatgtctcctgaggaatgatacccacggatacccacaattgtcctctggtctccgtgtgcaatacaaacccatgtctgaatatttgcaacagggtaaacattagagtttgatgttcagaattagactagattccctcatctagtaaagctgtgctttggccctcccatctgtcttatttttctactggtgtgctaaggcaccatgaccaaggcaacttagagaagaagaaacagtttattgagggtttatagttatagagggtaaggcaaggacttggtagcaggcaggcaggcaggcatggtactggtgtagtagctgggagcttgtatcttgagacacggttacaaagctgagagatagctaagtgggcctggtgtgagcttttgaaacctcaaagctgtccccagtgaaatgcctccatcaacaaggccacacctaacccttcccaaacagttctaccaactgggaaccaagcattcatatgagcctcaggggagcagtctcattcaagtaagtactcagtacactgccccatgggcagaagtcctctaaacggttactaatgtgtgtgtgtatatccctcaccatacttagaaggaaacaagccatcccaaaatggatagcatgactcagaaagttcctgtgtacttcacccagagcaaatgtggatacggtgggaaacagaggacagtgataggacacaaaggctgtgctgtctcagtttctagttcagatggagacataaaccaacacacataggaaagatacactccactggacagtgggagcccatgcacaaaggttctttggctcatttagtctatgctgtttctattcttcgatgacagcagtttcttattattgggaaataagatcagtagatgagctttgtttctgccctgggtgagagtttatttaggaacacacatgtgatcacactaagacaaccactgatggcctagaacaaagtcagagcactgtgcgttgtggatcttaggccattcatgatgattaaagcatccatcctattaaaatgtgttagtccatttttggggttatgtttactatacaaaggtggaaggggttatctggccccatcttacaggtaactgtgtcccttttgtggatataaaaaccatcagatactgcaattttatttttgtaaaaagcaactgtttttttttaagacttattttatttttgattatgtgtctgagggagcagtatgcacatctgcatgcaggtgcctgtggaagcctgtggagacatcagatcacctgaagctggagtttcaggcagttttatgccaccagacactggtgctgagaatagagtctcctgcaaaagcagtatattttattaatctgtgagccatctctccagccaaaagcaacctttaaaagctgtggtttatgtgccatttaattcatccacttagagggtacacttcaatagttttttttaaaaatatgcttacagatctgtgggcacatatgatccaattttagaacccttttagcactacagatattaaatacttactccctattctccccagcccccagctccagtccctggcatccacaaatccccttcctgccatctatagattcacctcttctagactttacactgaaatggtattacacaacatgtggtcttttgtcttttgcttgccgtgtgtctgtgaggttcatctgtgttgagcatgaaaggataacagatttacccatgaatatgcctgtcgcctaaaatagcaacactttcacactagaagcaatttccttctttcttcttcccaagagggacattattgcagcctgctagttttctcctgtgtcttttttcgtgtttctcaagtagatgaagggactggttacttttatttttttaatcattcatacttttatacttttctcccctgctttgtcagtttcctaaatgagtgaatactgtatttggtgatccccaatcagaaagaccaaaataatttaaaataatctcgtctctatatcactaaggtatccttttccacttgggccatgcagagaaataagcatgccttgattgaccccaccccaccccaacccccagtggtgacaaggacctccccagcggctcaaccatttgaataaaaaggacacttgagcccattttgcacaaatctaagatgagcaagtggcagtgtcacctgtaaacatgtgcctggagcacggaacgacctgagtaggcagaaaaaggtggaagtaatttatgatttttcttttaaaggttgccatttcccccacctttctcactttccaacaatattatattctggtgtgatatgttgtagacaaaaaaagctttaagcttttattccccagttgttttggtgattaaatcattttgggggaactgcaacagtgactctcattcactgctcccttggtgacagtgttttttttctgtaaaaagcgcctgctgttccctctgtctctgctcattttcataggaatctggcaccttagaatcccaggctgcctgcagtcaaatgcttgctagggaggggagccagtgggtgggggaacctgcaagaaatcaactccaaatttaataggactaagctcctacaccatgcctgattagcagctaggtctcatccttacccctccaggaataaggaaggttgcagaagtccctgaaaggtatttgctgagcctcttgtgaaccgtgggttggctcacctgaactttagtagatattctttagcgacatatttgggctttggtcctctctcttttatctctccacaaaagtcttggcaaactgatgtttatgcaaccagtaaggcctctggggctgagggggtgggaagccagtgggtggcggaacctgcaagaaatccgccccaaatttaaggaagcataggaataagctcctaccctatgtctgccttgtggctaggtccttagttcattgtctcttaggtatcccagattctcttgagagtagaaggtggaacatagtacctcctgattaacaaatccgagaggtgctaatctcatgaattctcccggactatggttatatatagctcagtgatctcatgtagcttaggctggctggaagctagttttgagctcactatgaagcaaaggatgaccctgaacttcttggttttcctgctttcatcttccaagtgctgcgattacaagaatgaatgctgccatgtctagttcatgtggtgctagggatcaaccctgaggctttgtgcatgttaagacaagcactctactaactgagctctagctctagccctgaccctgactcaaaagaatagggggggaggaaggaaggaaggaaggaaggaagggagggagggagggagggagggagggagggagggagggaggaaggatgttgagaacaaaagccaaggccaacaggtgagttgggattaggaaaagtccttttcatagcaaaggggatgtggaagaagagaagttgacaggtaagtagggaaatttgagacaaagaaaaaagaaaaaaatctgtggaccagggcatggcaagaaacgcagagagcaaatgttcataaagagaggtgggcaggaggcagaccatggtctcaagactcatcagagagataaggcaatatcctgaggagcacccatctgaggggcgttgagcaagtgggtttcatttctctgcattcacagatggaggatagatgtgtgcaactatctttagcagtgaggcatgctgggtagtgctaagagcgggcggggtctgtggaatggagaggagaaaccactccttattaccacgtcattttacttttgattatcttcattgtgatttagtgttctagtttgtgaatttatcactatgtatcttgcctcttgacggtcacacaagtacttccagttgaagagtaggcattacaaggtctgcttccatgaatattctagggcacatttttattccaggaaaaaatatatgaaagcatttctaattatgaatggaattggtggtttatggggaacacatatgctcagccttggaataaattaccaaaaccaaagaggctagactcccttctaccgatcaacagaagcatataagagttggcactgttctctactctaccaacttgtggttgggtcctgtttagaataataagaggcatctacatgtagagctctaggaagccattcaatgcaggatctaaaccttggctttagcaatgtctgtgcggtacttggagtaagctaagctctcaaagaaaaccaagatttatcggaatggtggacactgaaagtagacaggaaaggctgacaatacctagtgtgcagtgtgcagatggaagggcagtgctggggagaatccattgcatttggaaagaagaagccctctgcgatttcttttgctaatgcaggccttttcactgtagtacttgcttgtggtggtttgaatgaaaatggtccccacaggctatttttgaaaacttgatccccagttggtgaaactgtttggaaaggattaggaagtgtggccttgctggatgaggtctgtcaatggcggaaggctttgaagtttcccagtgtgcctctctctgtctcctacttattgattgaaaaatgagctttcagctgtcatgcctttgctctgccatccagaattctaatcacccaaaaccatatagcctaattaaatactgtttttataagttaccttggtcatggtactttaggatatcaatagttaagaaactaagacattggttcacttgctcaacttaaccaaaacaccacagacgggcttgcatatgacaacagttctagaggatcaaatgtccctgatcaaatgccctagcaggttctgtgtctgatgagggctgctggttcatgggtggtgctttttctcagtgtccttacaggtggaaggtatccagctttcttggaccttatattaaagcacgcattccattgatgtgagtagatagcttagtcagagccccaaagtgatttaagcacctccaaaaccctccgtctccggatgctcccccattggtgaacagatttcaacatagcaattgagcaggaggaaaggaagccaaattatttgatcacagccagtactttggtgaacacccaaacccagcatggagctgaatatctgtaatctcagtatccagcaggtggatattggggaattaagacttcaaggccagacttggctacatagtaagtttgatgccatcctgggctatatgagatcctgtttccaaaacccccaaatagaaacaataaaaaaatggcagtccttcatgttcactgctaccctagaaggtcagttttgcttgtaacagatgactaacagaggaacaaggtcccggaagagctaccagtatgctggctgccaatgaagctgctgaagtcttagtagatttaggagctatggtcctgacttccatcacagccccagcaccaccatgggcactgcccagcagtctatcttcttttaggtcttcaggtgtccctgggtagagaacaaggcttctgcttgcatagggctgatgccccagtacagtgacagtctcacaatgagtgcagcaatgtggccacagaacggggaaatgtgtgttctttaactagtagcttttataatcatgataaaaagataagtgtctactctcaagctgaaagcttttcacaggcatctgattctcttgctaaatgacaaagtggttagaggagggacctacagctttcattgtctacactcaggtttcttttgagaattttacagtaggtatgtattgttttctagtcaacacagaaataaaaggatttgttttgttgaaaagaagtgggggttttggtactgatgaggggaaattgatttatgttacttattcattctcaggttcatggctgagactccttatgacaaatgatagattaataaaagcatgcaaatgctggagctctgctggcggagtacctgatatgcaaggatgaagatctctgttcaatccccagaaatcaaataaaaaagctgggcatagtgaggaagaggagatgggaggattcctgtggctggctggacagctaacctagcctattcatctatttccaggccactaagggatggtaccttaaaaaataacaataataataaaaaataacaataataataaataaaaaaggtagctggttcctgaggagcatctaaggatatcctttaactccacgtgcacatacactgtatacacaggaacacatacaagcatgcagatttacctatcaagttttaccaaaaaaaaaaaaaaaaaaaaaaaagaacactttattcactgttggtgggtatgtaaactggcatatgtagccactatgaaaatcagcacagaggttcccttcccactccaacaaaacaaaacaaaacaaaacaaaacaaaacaaaacaaaacaaaacaaaaccctctagaactagaactagaactactgcacgatccaggtttaccactcctaggtatttactcaaaggactctatacgtcaacctgtgacagaggcatcatatacaagcagggagtggtggcacctgcctttaatcccacccctcaggaggcagagtcaggtagatctctgtgagttcgaggccagtttggtctacatagtgagttctagtacagccataagaccatatagccatatggaggggggattgtgagcatagagtatgaatgttcttgagagaattattaaatgaattggaattattatacactgtcttctttcataggaaaaatgaacagaaagggagagatctttgggtggggctaacagcatacatgacatgaaagcagaaggggattagttattggaaggcagggagggacccaggaggatgaagggaagagaatgcaagggaaaggagtaaaggaggaggaggtagaggtacacactattaattccagcacttgtgaggaggggacagagctctgtgagttcaaggtcagccccctctgcatagtcagttccaggatagccaatggctacataatgagaccctgtgtcagagaaggtggccggcgagggatattgatgcttacagtttactttagccaccacacagctgaatgagttaaacctgttcctgctacttttgcactttcaatgctcccagattacttacatggaatttatattttattgtggtttaatagctcctgtacatcatagacaaacctcaagaaaaattttcaaccaatagtccaggcaaaaataacctctttttctttctttctttctttctttttttttttttttttttggttttttgaaacagggtttctctgtatagccctggctgtcctggaactcactttgtacaccaggctggcctcgaactcagaaatccacctgcctctgcctcccgagtgctcggattaaaggcgtgcaccaccaccgtcccgcaaaaaataacctgtttttgttgttttaattatttttaagattttatgtgtatgggtgtctgtctgtatgtatgtctgtgtaccacttgtatgcttggtgcccaagaaggacagaacagatcatagggtttcctgggataagagttataggagttatagatgactgtaagccaccaagtggacgctgggaattgaaccttggttagctggaagagtgtccagtatttttaattccagtccccgttgtttgtctatgaagattttgcttggtagtccagtctggctttaagaaacagggtctcatgcatccctggcttgctcagacttccatgcagctgaggatggctttagagtaacaaccctcctgccttttcctcgtagagtgctgagattacagtcctgtgccaccagcagacttctcctaacaagaatgtggcacagggaggcaactgggaatcaaacaggaaggaggagtaaaaggaaggggaggaaggagaggagaagtggcaggaggagaagaaaaaggaggcggagaaaaggtggtagtggtggaggaagaggaggaggaggaggaggaggaggagggggacttaatcagtaaaggaaaaaggctgagctcagtccttggaacctacatggtaggagagaatgagacttctgcaaagtttcctctgatccccacactggagcaatggtgccatcacatcactctcccacttcacccaactcctcacaaaaataaaaaacaaaaacaaaacaacagacaaacaaatacataaataaatgtagtttaaaaaagaaagctgtagccgggcgtggtggcacacacttttaatcccggcacttgggaggcagaggcaagcggatttctgagttcgaggccagcttggtctacaaagtgagttccaggacagccagggctacacagagaaaccctgtcttgaaaaaccaaaagaaaaaaagaaagctgtactgcaccctgctttgctatattaatatattttccataattctataagaaaaaacaacagtcattgccatccttttcctccctccagaatgagctccttaatctctatggcattgttttcattttgccttctttcctttcttaatttcattttttccctctcttgttcttttgctcagccacattgggattgtcatcgacagaggtatgttacagtaagaagggtggaattttcatcggtgttgcttttgaagtaaaactaatatatgagtctagcactattggggggaagagtgctgagggtgaagccaagggccttgggcatgctaggcacgtgattcacactgataccctactcctgaagcctgagagcctttttcaaatgtctgttgttttagttgggtgttgggtgtgggcatgagtggaaaggcaggtcttcctattgttctatccctccttgccttaattcaggctctctcactaaactggaagcttgcttttgtggttaggtgggctggccatgagttacccaaatcacccttctctatcccctccccccctaaactatggccacatcaagcagccatgcccagctttctgcctgggctctggagatttgagctcaggtgctcatatttgcacagcaaaggctcttacccacttagccatctccccagcccctttcaaatgtttttttttttaagttttacactgaacttaggcctatcactccagcatgcagtaaactgaggcactcaagtctagttatcctgggctacaaagtgagacattgactaaaaggaaaaagagaaaaggaaggaagggagggagggaggaagaaaggaaggaaggaaggaaggaaggaaggaaggaaggaaggaaggaaggaagggagggagggagggagggagggagggagaaaggagagagagagaaagaggacaaagaaggagggaaagatggatggatggagggagggagggagggagggagagaaagaggggggagttcagtggagaagctagggatatggctcagttggcagagtgcttatctagcatacatgatagtgaatgcctataatctcagaactctagaggcatcattccaaggttttactttgactccatagagtttaaggccagcttgggacacaagagactgtgtctcaaaacaaggaaataaaaacaaaaatctaaaaaacacccacccagacctattttaggcaccttttttgtccatgctaggcaagtgatttaacacttagctgcatccataggaagcttgctggacttctttgtttttgggacaggagttttgtatgtagcccagataccagacccagttacattggcatttgttttgctattgttattgctttttgatgtcattgttgcttttttttttttttttttttttttttttttggcaagttctcctgtagcccaggcttgcctggaactctggaacttgataggtagctgatgataactttgtactcttgatcctcctatccctatcttccaagtgctgggattacagtcacgtactactctagttttaaaattggatgccttagataggatcctccagggagcataaagagtccaatcttgtactggaactccatctccaagaaggtaaacattatccttgtgtacataggtagccctaggaataatcagttggtgcctatagtgagaagcatttttttttttatttagatgagcagggcatggtggaacatgtctttaattctagcatttgggacatagaggcaggaggatcaaaaggctcaaggccattcttggctacacagagagttggaggttagccagcctgtgctgaatgagacccagcctgaaacaaaaagggggaggtgggagatagaaggatggctcctgtggtaaatccagagactcataaaaaatgctgggcatggtggcaggagtttgtaatcccagtgtcggggaggtgaagacaagagaatccccagggcatgctggccaactaactagtctagcctaattggtgagctccaggacagtaagataccctgcttcaaagaaggcacatgggattcctgaggatgccacccaaaggtgtcctctagcatcctcacatgagcatgcaagaacatgtgcacctgaatgtaacatgtgcgcacacacacacacacacacacacacacacacacacacacacacatttttaaaaagtaatatagagctggagtgtacctttgttgatagaacacttgtttaggattcgtgaaggtcttgatttgatcctaagcaccatgtaaactgggcacccatctagaagcccagcactcagaggtggagacaggaggtcaggagttcaacaaggtcattctctgctacacagtgagtttaaaatcggcctgggatacacgagagagaccctgtgtaagagcagtagcagcagcaagaactcaagctgaaaaggaacatgcagtgtaagacaaagggccactgtgtgcatagagccagcaacctcacactgtaatgaacgggtctgacctttgcaagtaagcttcttgtgatgctctggttgagcctttgactacgacttttgtgacttgtgctcctctggatgcttgcaggatgagggtgaggacccctggtaccagaaagcatgcaagtgtgattgccaggtaggagccaatgctctgtggtctgctggagctacctccttagactgta

SEQ ID NO: 25 - DNA, 3670 bp, Artificial Sequence
  recombinant or synthetic polynucleotide
aagaactaaatgaaataagatgcttaagttaatcgcctgctcctatgccagctctccacttcacttagatcttgctgtgaccaaggacaaggagaaaatgggtaccgatttaaatgatccagtggtcctgcagaggagagattgggagaatcccggtgtgacacagctgaacagactagccgcccaccctccctttgcttcttggagaaacagtgaggaagctaggacagacagaccaagccagcaactcagatctttgaacggggagtggagatttgcctggtttccggcaccagaagcggtgccggaaagctggctggagtgcgatcttcctgaggccgatactgtcgtcgtcccctcaaactggcagatgcacggttacgatgcgcccatctacaccaacgtgacctatcccattacggtcaatccgccgtttgttcccacggagaatccgacgggttgttactcgctcacatttaatgttgatgaaagctggctacaggaaggccagacgcgaattatttttgatggcgttaactcggcgtttcatctgtggtgcaacgggcgctgggtcggttacggccaggacagtcgtttgccgtctgaatttgacctgagcgcatttttacgcgccggagaaaaccgcctcgcggtgatggtgctgcgctggagtgacggcagttatctggaagatcaggatatgtggcggatgagcggcattttccgtgacgtctcgttgctgcataaaccgactacacaaatcagcgatttccatgttgccactcgctttaatgatgatttcagccgcgctgtactggaggctgaagttcagatgtgcggcgagttgcgtgactacctacgggtaacagtttctttatggcagggtgaaacgcaggtcgccagcggcaccgcgcctttcggcggtgaaattatcgatgagcgtggtggttatgccgatcgcgtcacactacgtctgaacgtcgaaaacccgaaactgtggagcgccgaaatcccgaatctctatcgtgcggtggttgaactgcacaccgccgacggcacgctgattgaagcagaagcctgcgatgtcggtttccgcgaggtgcggattgaaaatggtctgctgctgctgaacggcaagccgttgctgattcgaggcgttaaccgtcacgagcatcatcctctgcatggtcaggtcatggatgagcagacgatggtgcaggatatcctgctgatgaagcagaacaactttaacgccgtgcgctgttcgcattatccgaaccatccgctgtggtacacgctgtgcgaccgctacggcctgtatgtggtggatgaagccaatattgaaacccacggcatggtgccaatgaatcgtctgaccgatgatccgcgctggctaccggcgatgagcgaacgcgtaacgcgaatggtgcagcgcgatcgtaatcacccgagtgtgatcatctggtcgctggggaatgaatcaggccacggcgctaatcacgacgcgctgtatcgctggatcaaatctgtcgatccttcccgcccggtgcagtatgaaggcggcggagccgacaccacggccaccgatattatttgcccgatgtacgcgcgcgtggatgaagaccagcccttcccggctgtgccgaaatggtccatcaaaaaatggctttcgctacctggagagacgcgcccgctgatcctttgcgaatacgcccacgcgatgggtaacagtcttggcggtttcgctaaatactggcaggcgtttcgtcagtatccccgtttacagggcggcttcgtctgggactgggtggatcagtcgctgattaaatatgatgaaaacggcaacccgtggtcggcttacggcggtgattttggcgatacgccgaacgatcgccagttctgtatgaacggtctggtctttgccgaccgcacgccgcatccagcgctgacggaagcaaaacaccagcagcagtttttccagttccgtttatccgggcaaaccatcgaagtgaccagcgaatacctgttccgtcatagcgataacgagctcctgcactggatggtggcgctggatggtaagccgctggcaagcggtgaagtgcctctggatgtcgctccacaaggtaaacagttgattgaactgcctgaactaccgcagccggagagcgccgggcaactctggctcacagtacgcgtagtgcaaccgaacgcgaccgcatggtcagaagccgggcacatcagcgcctggcagcagtggcgtctggcggaaaacctcagtgtgacgctccccgccgcgtcccacgccatcccgcatctgaccaccagcgaaatggatttttgcatcgagctgggtaataagcgttggcaatttaaccgccagtcaggctttctttcacagatgtggattggcgataaaaaacaactgctgacgccgctgcgcgatcagttcacccgtgcaccgctggataacgacattggcgtaagtgaagcgacccgcattgaccctaacgcctgggtcgaacgctggaaggcggcgggccattaccaggccgaagcagcgttgttgcagtgcacggcagatacacttgctgatgcggtgctgattacgaccgctcacgcgtggcagcatcaggggaaaaccttatttatcagccggaaaacctaccggattgatggtagtggtcaaatggcgattaccgttgatgttgaagtggcgagcgatacaccgcatccggcgcggattggcctgaactgccagctggcgcaggtagcagagcgggtaaactggctcggattagggccgcaagaaaactatcccgaccgccttactgccgcctgttttgaccgctgggatctgccattgtcagacatgtataccccgtacgtcttcccgagcgaaaacggtctgcgctgcgggacgcgcgaattgaattatggcccacaccagtggcgcggcgacttccagttcaacatcagccgctacagtcaacagcaactgatggaaaccagccatcgccatctgctgcacgcggaagaaggcacatggctgaatatcgacggtttccatatggggattggtggcgacgactcctggagcccgtcagtatcggcggaattccagctgagcgccggtcgctaccattaccagttggtctggtgtcaaaaataataataaccgggcaggggggatctaagctctagataagtaatgatcataatcagccatatcacatctgtagaggttttacttgctttaaaaaacctcccacacctccccctgaacctgaaacataaaatgaatgcaattgttgttgttaacttgtttattgcagcttataatggttacaaataaagcaatagcatcacaaatttcacaaataaagcatttttttcactgcattctagttgtggtttgtccaaactcatcaatgtatcttatcatgtctggatcccccggctagagtttaaacactagaactagtggatccccgggctcgataactataacggtcctaaggtagcgactcgacataacttcgtataatgtatgctatacgaagttatgctagcttccaggtgagtggctcaacgccctagcattcctccttccaactcttaatccctctgctttctctcaagttggcttgtgagcttcacatctcaccgtggc

SEQ ID NO: 26 - DNA, 5987 bp, Artificial Sequence
  recombinant or synthetic polynucleotide
gcatgcaagaacatgtgcacctgaatgtaacatgtgcgcacacacacacacacacacacacacacacacacacacacacacatttttaaaaagtaatatagagctggagtgtacctttgttgatagaacacttgtttaggattcgtgaaggtaaactgggcacccatctagaagcccagcactcagaggtggagacaggaggtcaggagttcaacaaggtcattctctgctacacagtgagtttaaaatcggcctgggatacacgagagagaccctgtgtaagagcagtagcagcagcaagaactcaagctgaaaaggaacatgcagtgtaagacaaagggccactgtgtgcatagagccagcaacctcacactgtaatgaacgggtctgacctttgcaagtaagcttcttgtgatgctctggttgagcctttgactacgacttttgtgacttgtgctcctctggatgcttgcaggatgagggtgaggacccctggtaccagaaagcatgcaagtgtgattgccaggtaggagccaatgctctgtggtctgctggagctacctccttagacagtattccaggtgagtggctcaacgccctagcattcctccttccaactcttaatccctctgctttctctcaagttggcttgtgagcttcacatctcaccgtggccactgctccaacattctgttcattatcaagtgccaggctctctccctccctggcttgcctgagatggtcaggtaagacccctcgagataacttcgtataatgtatgctatacgaagttatatgcatgccagtagcagcacccacgtccaccttctgtctagtaatgtccaacacctccctcagtccaaacactgctctgcatccatgtggctcccatttatacctgaagcacttgatggggcctcaatgttttactagagcccacccccctgcaactctgagaccctctggatttgtctgtcagtgcctcactggggcgttggataatttcttaaaaggtcaagttccctcagcagcattctctgagcagtctgaagatgtgtgcttttcacagttcaaatccatgtggctgtttcacccacctgcctggccttgggttatctatcaggacctagcctagaagcaggtgtgtggcacttaacacctaagctgagtgactaactgaacactcaagtggatgccatctttgtcacttcttgactgtgacacaagcaactcctgatgccaaagccctgcccacccctctcatgcccatatttggacatggtacaggtcctcactggccatggtctgtgaggtcctggtcctctttgacttcataattcctaggggccactagtatctataagaggaagagggtgctggctcccaggccacagcccacaaaattccacctgctcacaggttggctggctcgacccaggtggtgtcccctgctctgagccagctcccggccaagccagcaccatgggaacccccaagaagaagaggaaggtgcgtaccgatttaaattccaatttactgaccgtacaccaaaatttgcctgcattaccggtcgatgcaacgagtgatgaggttcgcaagaacctgatggacatgttcagggatcgccaggcgttttctgagcatacctggaaaatgcttctgtccgtttgccggtcgtgggcggcatggtgcaagttgaataaccggaaatggtttcccgcagaacctgaagatgttcgcgattatcttctatatcttcaggcgcgcggtctggcagtaaaaactatccagcaacatttgggccagctaaacatgcttcatcgtcggtccgggctgccacgaccaagtgacagcaatgctgtttcactggttatgcggcggatccgaaaagaaaacgttgatgccggtgaacgtgcaaaacaggtaaatataaaatttttaagtgtataatgatgttaaactactgattctaattgtttgtgtattttaggctctagcgttcgaacgcactgatttcgaccaggttcgttcactcatggaaaatagcgatcgctgccaggatatacgtaatctggcatttctggggattgcttataacaccctgttacgtatagccgaaattgccaggatcagggttaaagatatctcacgtactgacggtgggagaatgttaatccatattggcagaacgaaaacgctggttagcaccgcaggtgtagagaaggcacttagcctgggggtaactaaactggtcgagcgatggatttccgtctctggtgtagctgatgatccgaataactacctgttttgccgggtcagaaaaaatggtgttgccgcgccatctgccaccagccagctatcaactcgcgccctggaagggatttttgaagcaactcatcgattgatttacggcgctaaggatgactctggtcagagatacctggcctggtctggacacagtgcccgtgtcggagccgcgcgagatatggcccgcgctggagtttcaataccggagatcatgcaagctggtggctggaccaatgtaaatattgtcatgaactatatccgtaacctggatagtgaaacaggggcaatggtgcgcctgctggaagatggcgattaggcggccggccgctaatcagccataccacatttgtagaggttttacttgctttaaaaaacctcccacacctccccctgaacctgaaacataaaatgaatgcaattgttgttgttaacttgtttattgcagcttataatggttacaaataaagcaatagcatcacaaatttcacaaataaagcatttttttcactgcattctagttgtggtttgtccaaactcatcaatgtatcttatcatgtctggatcccccggctagagtttaaacactagaactagtggatcccccgggatcatggcctccgcgccgggttttggcgcctcccgcgggcgcccccctcctcacggcgagcgctgccacgtcagacgaagggcgcagcgagcgtcctgatccttccgcccggacgctcaggacagcggcccgctgctcataagactcggccttagaaccccagtatcagcagaaggacattttaggacgggacttgggtgactctagggcactggttttctttccagagagcggaacaggcgaggaaaagtagtcccttctcggcgattctgcggagggatctccgtggggcggtgaacgccgatgattatataaggacgcgccgggtgtggcacagctagttccgtcgcagccgggatttgggtcgcggttcttgtttgtggatcgctgtgatcgtcacttggtgagtagcgggctgctgggctggccggggctttcgtggccgccgggccgctcggtgggacggaagcgtgtggagagaccgccaagggctgtagtctgggtccgcgagcaaggttgccctgaactgggggttggggggagcgcagcaaaatggcggctgttcccgagtcttgaatggaagacgcttgtgaggcgggctgtgaggtcgttgaaacaaggtggggggcatggtgggcggcaagaacccaaggtcttgaggccttcgctaatgcgggaaagctcttattcgggtgagatgggctggggcaccatctggggaccctgacgtgaagtttgtcactgactggagaactcggtttgtcgtctgttgcgggggcggcagttatggcggtgccgttgggcagtgcacccgtacctttgggagcgcgcgccctcgtcgtgtcgtgacgtcacccgttctgttggcttataatgcagggtggggccacctgccggtaggtgtgcggtaggcttttctccgtcgcaggacgcagggttcgggcctagggtaggctctcctgaatcgacaggcgccggacctctggtgaggggagggataagtgaggcgtcagtttctttggtcggttttatgtacctatcttcttaagtagctgaagctccggttttgaactatgcgctcggggttggcgagtgtgttttgtgaagttttttaggcaccttttgaaatgtaatcatttgggtcaatatgtaattttcagtgttagactagtaaattgtccgctaaattctggccgtttttggcttttttgttagacgtgttgacaattaatcatcggcatagtatatcggcatagtataatacgacaaggtgaggaactaaaccatgaaaaagcctgaactcaccgcgacgtctgtcgagaagtttctgatcgaaaagttcgacagcgtgtccgacctgatgcagctctcggagggcgaagaatctcgtgctttcagcttcgatgtaggagggcgtggatatgtcctgcgggtaaatagctgcgccgatggtttctacaaagatcgttatgtttatcggcactttgcatcggccgcgctcccgattccggaagtgcttgacattggggaattcagcgagagcctgacctattgcatctcccgccgtgcacagggtgtcacgttgcaagacctgcctgaaaccgaactgcccgctgttctgcagccggtcgcggaggccatggatgcgattgctgcggccgatcttagccagacgagcgggttcggcccattcggaccgcaaggaatcggtcaatacactacatggcgtgatttcatatgcgcgattgctgatccccatgtgtatcactggcaaactgtgatggacgacaccgtcagtgcgtccgtcgcgcaggctctcgatgagctgatgctttgggccgaggactgccccgaagtccggcacctcgtgcacgcggatttcggctccaacaatgtcctgacggacaatggccgcataacagcggtcattgactggagcgaggcgatgttcggggattcccaatacgaggtcgccaacatcttcttctggaggccgtggttggcttgtatggagcagcagacgcgctacttcgagcggaggcatccggagcttgcaggatcgccgcggctccgggcgtatatgctccgcattggtcttgaccaactctatcagagcttggttgacggcaatttcgatgatgcagcttgggcgcagggtcgatgcgacgcaatcgtccgatccggagccgggactgtcgggcgtacacaaatcgcccgcagaagcgcggccgtctggaccgatggctgtgtagaagtactcgccgatagtggaaaccgacgccccagcactcgtccgagggcaaaggaatagggggatccgctgtaagtctgcagaaattgatgatctattaaacaataaagatgtccactaaaatggaagtttttcctgtcatactttgttaagaagggtgagaacagagtacctacattttgaatggaaggattggagctacgggggtgggggtggggtgggattagataaatgcctgctctttactgaaggctctttactattgctttatgataatgtttcatagttggatatcataatttaaacaagcaaaaccaaattaagggccagctcattcctcccactcatgatctatagatctatagatctctcgtgggatcattgtttttctcttgattcccactttgtggttctaagtactgtggtttccaaatgtgtcagtttcatagcctgaagaacgagatcagcagcctctgttccacatacacttcattctcagtattgttttgccaagttctaattccatcagacctcgacctgcagcccctagataacttcgtataatgtatgctatacgaagttatgctaggtaactataacggtcctaaggtagcgagctagcagcgtgagggaagtcccttcctcttaggtatcagaggaaatgtgtgtgtgtgtgtgtgtgtgtgtgtttctatatcctgtggagtcatgctgtctctaaatcagtaatgaggatatggagggcaagaatttagtaaaacaagtcgcttctagaagctaaattactgtcatttcatggattggcagaaaactgggcaccca

SEQ ID NO: 27 - DNA, 1033 bp, Artificial Sequence
  recombinant or synthetic polynucleotide
gcatgcaagaacatgtgcacctgaatgtaacatgtgcgcacacacacacacacacacacacacacacacacacacacacacatttttaaaaagtaatatagagctggagtgtacctttgttgatagaacacttgtttaggattcgtgaaggtaaactgggcacccatctagaagcccagcactcagaggtggagacaggaggtcaggagttcaacaaggtcattctctgctacacagtgagtttaaaatcggcctgggatacacgagagagaccctgtgtaagagcagtagcagcagcaagaactcaagctgaaaaggaacatgcagtgtaagacaaagggccactgtgtgcatagagccagcaacctcacactgtaatgaacgggtctgacctttgcaagtaagcttcttgtgatgctctggttgagcctttgactacgacttttgtgacttgtgctcctctggatgcttgcaggatgagggtgaggacccctggtaccagaaagcatgcaagtgtgattgccaggtaggagccaatgctctgtggtctgctggagctacctccttagacagtattccaggtgagtggctcaacgccctagcattcctccttccaactcttaatccctctgctttctctcaagttggcttgtgagcttcacatctcaccgtggccactgctccaacattctgttcattatcaagtgccaggctctctccctccctggcttgcctgagatggtcaggtaagacccctcgagataacttcgtataatgtatgctatacgaagttatgctaggtaactataacggtcctaaggtagcgagctagcagcgtgagggaagtcccttcctcttaggtatcagaggaaatgtgtgtgtgtgtgtgtgtgtgtgtgtttctatatcctgtggagtcatgctgtctctaaatcagtaatgaggatatggagggcaagaatttagtaaaacaagtcgcttctagaagctaaattactgtcatttcatggattggcagaaaactgggcaccca

SEQ ID NO: 28 - DNA, 5629 bp, Artificial Sequence
  recombinant or synthetic polynucleotide
aagagctcatttgttaaacatgccagggaagtctttcctaaggaaaagaattaagagtcgggctatgtctgaaggcccagatacctcttgatgctaggtaacccttcaaaactcagcacctgttggctttttacagacatagataagaggatggctcctggtaatttggtgtgttcctggcaggtgtgcttggctttccaagtatcaggacagcagccagtggttacagatagatttgaaggagatcaaggtgatttcggggatcctgacccaaggatgctgtgacatagacgagtgggtgaccaagtacagtgtgcagtataggactgatgagcgcctgaactggatctactataaggatcagaccggaaacaatcgggtaagtgggggtcactccgagtcagcttcagctcacactgcggagacacactccatccctatgttcctgctgtccgcgtctgtctgagcattgacccctctacatgctgggtcatctgctcgagataacttcgtataatgtatgctatacgaagttatatgcatgccagtagcagcacccacgtccaccttctgtctagtaatgtccaacacctccctcagtccaaacactgctctgcatccatgtggctcccatttatacctgaagcacttgatggggcctcaatgttttactagagcccacccccctgcaactctgagaccctctggatttgtctgtcagtgcctcactggggcgttggataatttcttaaaaggtcaagttccctcagcagcattctctgagcagtctgaagatgtgtgcttttcacagttcaaatccatgtggctgtttcacccacctgcctggccttgggttatctatcaggacctagcctagaagcaggtgtgtggcacttaacacctaagctgagtgactaactgaacactcaagtggatgccatctttgtcacttcttgactgtgacacaagcaactcctgatgccaaagccctgcccacccctctcatgcccatatttggacatggtacaggtcctcactggccatggtctgtgaggtcctggtcctctttgacttcataattcctaggggccactagtatctataagaggaagagggtgctggctcccaggccacagcccacaaaattccacctgctcacaggttggctggctcgacccaggtggtgtcccctgctctgagccagctcccggccaagccagcaccatgggaacccccaagaagaagaggaaggtgcgtaccgatttaaattccaatttactgaccgtacaccaaaatttgcctgcattaccggtcgatgcaacgagtgatgaggttcgcaagaacctgatggacatgttcagggatcgccaggcgttttctgagcatacctggaaaatgcttctgtccgtttgccggtcgtgggcggcatggtgcaagttgaataaccggaaatggtttcccgcagaacctgaagatgttcgcgattatcttctatatcttcaggcgcgcggtctggcagtaaaaactatccagcaacatttgggccagctaaacatgcttcatcgtcggtccgggctgccacgaccaagtgacagcaatgctgtttcactggttatgcggcggatccgaaaagaaaacgttgatgccggtgaacgtgcaaaacaggtaaatataaaatttttaagtgtataatgatgttaaactactgattctaattgtttgtgtattttaggctctagcgttcgaacgcactgatttcgaccaggttcgttcactcatggaaaatagcgatcgctgccaggatatacgtaatctggcatttctggggattgcttataacaccctgttacgtatagccgaaattgccaggatcagggttaaagatatctcacgtactgacggtgggagaatgttaatccatattggcagaacgaaaacgctggttagcaccgcaggtgtagagaaggcacttagcctgggggtaactaaactggtcgagcgatggatttccgtctctggtgtagctgatgatccgaataactacctgttttgccgggtcagaaaaaatggtgttgccgcgccatctgccaccagccagctatcaactcgcgccctggaagggatttttgaagcaactcatcgattgatttacggcgctaaggatgactctggtcagagatacctggcctggtctggacacagtgcccgtgtcggagccgcgcgagatatggcccgcgctggagtttcaataccggagatcatgcaagctggtggctggaccaatgtaaatattgtcatgaactatatccgtaacctggatagtgaaacaggggcaatggtgcgcctgctggaagatggcgattaggcggccggccgctaatcagccataccacatttgtagaggttttacttgctttaaaaaacctcccacacctccccctgaacctgaaacataaaatgaatgcaattgttgttgttaacttgtttattgcagcttataatggttacaaataaagcaatagcatcacaaatttcacaaataaagcatttttttcactgcattctagttgtggtttgtccaaactcatcaatgtatcttatcatgtctggatcccccggctagagtttaaacactagaactagtggatcccccgggatcatggcctccgcgccgggttttggcgcctcccgcgggcgcccccctcctcacggcgagcgctgccacgtcagacgaagggcgcagcgagcgtcctgatccttccgcccggacgctcaggacagcggcccgctgctcataagactcggccttagaaccccagtatcagcagaaggacattttaggacgggacttgggtgactctagggcactggttttctttccagagagcggaacaggcgaggaaaagtagtcccttctcggcgattctgcggagggatctccgtggggcggtgaacgccgatgattatataaggacgcgccgggtgtggcacagctagttccgtcgcagccgggatttgggtcgcggttcttgtttgtggatcgctgtgatcgtcacttggtgagtagcgggctgctgggctggccggggctttcgtggccgccgggccgctcggtgggacggaagcgtgtggagagaccgccaagggctgtagtctgggtccgcgagcaaggttgccctgaactgggggttggggggagcgcagcaaaatggcggctgttcccgagtcttgaatggaagacgcttgtgaggcgggctgtgaggtcgttgaaacaaggtggggggcatggtgggcggcaagaacccaaggtcttgaggccttcgctaatgcgggaaagctcttattcgggtgagatgggctggggcaccatctggggaccctgacgtgaagtttgtcactgactggagaactcggtttgtcgtctgttgcgggggcggcagttatggcggtgccgttgggcagtgcacccgtacctttgggagcgcgcgccctcgtcgtgtcgtgacgtcacccgttctgttggcttataatgcagggtggggccacctgccggtaggtgtgcggtaggcttttctccgtcgcaggacgcagggttcgggcctagggtaggctctcctgaatcgacaggcgccggacctctggtgaggggagggataagtgaggcgtcagtttctttggtcggttttatgtacctatcttcttaagtagctgaagctccggttttgaactatgcgctcggggttggcgagtgtgttttgtgaagttttttaggcaccttttgaaatgtaatcatttgggtcaatatgtaattttcagtgttagactagtaaattgtccgctaaattctggccgtttttggcttttttgttagacgtgttgacaattaatcatcggcatagtatatcggcatagtataatacgacaaggtgaggaactaaaccatgaaaaagcctgaactcaccgcgacgtctgtcgagaagtttctgatcgaaaagttcgacagcgtgtccgacctgatgcagctctcggagggcgaagaatctcgtgctttcagcttcgatgtaggagggcgtggatatgtcctgcgggtaaatagctgcgccgatggtttctacaaagatcgttatgtttatcggcactttgcatcggccgcgctcccgattccggaagtgcttgacattggggaattcagcgagagcctgacctattgcatctcccgccgtgcacagggtgtcacgttgcaagacctgcctgaaaccgaactgcccgctgttctgcagccggtcgcggaggccatggatgcgattgctgcggccgatcttagccagacgagcgggttcggcccattcggaccgcaaggaatcggtcaatacactacatggcgtgatttcatatgcgcgattgctgatccccatgtgtatcactggcaaactgtgatggacgacaccgtcagtgcgtccgtcgcgcaggctctcgatgagctgatgctttgggccgaggactgccccgaagtccggcacctcgtgcacgcggatttcggctccaacaatgtcctgacggacaatggccgcataacagcggtcattgactggagcgaggcgatgttcggggattcccaatacgaggtcgccaacatcttcttctggaggccgtggttggcttgtatggagcagcagacgcgctacttcgagcggaggcatccggagcttgcaggatcgccgcggctccgggcgtatatgctccgcattggtcttgaccaactctatcagagcttggttgacggcaatttcgatgatgcagcttgggcgcagggtcgatgcgacgcaatcgtccgatccggagccgggactgtcgggcgtacacaaatcgcccgcagaagcgcggccgtctggaccgatggctgtgtagaagtactcgccgatagtggaaaccgacgccccagcactcgtccgagggcaaaggaatagggggatccgctgtaagtctgcagaaattgatgatctattaaacaataaagatgtccactaaaatggaagtttttcctgtcatactttgttaagaagggtgagaacagagtacctacattttgaatggaaggattggagctacgggggtgggggtggggtgggattagataaatgcctgctctttactgaaggctctttactattgctttatgataatgtttcatagttggatatcataatttaaacaagcaaaaccaaattaagggccagctcattcctcccactcatgatctatagatctatagatctctcgtgggatcattgtttttctcttgattcccactttgtggttctaagtactgtggtttccaaatgtgtcagtttcatagcctgaagaacgagatcagcagcctctgttccacatacacttcattctcagtattgttttgccaagttctaattccatcagacctcgacctgcagcccctagataacttcgtataatgtatgctatacgaagttatgctaggtaactataacggtcctaaggtagcgagctagcttttccagatgtgatctgggagactagcagtttgtaaatgaatgtgggtcttttttgaaaaaaaggaaaaaaaagtaattttctagttctcactatcagc

SEQ ID NO: 29 - DNA, 675 bp, Artificial Sequence
  recombinant or synthetic polynucleotide
aagagctcatttgttaaacatgccagggaagtctttcctaaggaaaagaattaagagtcgggctatgtctgaaggcccagatacctcttgatgctaggtaacccttcaaaactcagcacctgttggctttttacagacatagataagaggatggctcctggtaatttggtgtgttcctggcaggtgtgcttggctttccaagtatcaggacagcagccagtggttacagatagatttgaaggagatcaaggtgatttcggggatcctgacccaaggatgctgtgacatagacgagtgggtgaccaagtacagtgtgcagtataggactgatgagcgcctgaactggatctactataaggatcagaccggaaacaatcgggtaagtgggggtcactccgagtcagcttcagctcacactgcggagacacactccatccctatgttcctgctgtccgcgtctgtctgagcattgacccctctacatgctgggtcatctgctcgagataacttcgtataatgtatgctatacgaagttatgctaggtaactataacggtcctaaggtagcgagctagcttttccagatgtgatctgggagactagcagtttgtaaatgaatgtgggtcttttttgaaaaaaaggaaaaaaaagtaattttctagttctcactatcagc

SEQ ID NO: 30 - DNA, 680 bp, Artificial Sequence
  recombinant or synthetic polynucleotide
ccagtagcagcacccacgtccaccttctgtctagtaatgtccaacacctccctcagtccaaacactgctctgcatccatgtggctcccatttatacctgaagcacttgatggggcctcaatgttttactagagcccacccccctgcaactctgagaccctctggatttgtctgtcagtgcctcactggggcgttggataatttcttaaaaggtcaagttccctcagcagcattctctgagcagtctgaagatgtgtgcttttcacagttcaaatccatgtggctgtttcacccacctgcctggccttgggttatctatcaggacctagcctagaagcaggtgtgtggcacttaacacctaagctgagtgactaactgaacactcaagtggatgccatctttgtcacttcttgactgtgacacaagcaactcctgatgccaaagccctgcccacccctctcatgcccatatttggacatggtacaggtcctcactggccatggtctgtgaggtcctggtcctctttgacttcataattcctaggggccactagtatctataagaggaagagggtgctggctcccaggccacagcccacaaaattccacctgctcacaggttggctggctcgacccaggtggtgtcccctgctctgagccagctcccggccaagccagcacc

SEQ ID NO: 31 - DNA, 1052 bp, Artificial Sequence
  recombinant or synthetic polynucleotide
tgccatcatcacaggatgtccttccttctccagaagacagactggggctgaaggaaaagccggccaggctcagaacgagccccactaattactgcctccaacagctttccactcactgcccccagcccaacatcccctttttaactgggaagcattcctactctccattgtacgcacacgctcggaagcctggctgtgggtttgggcatgagaggcagggacaacaaaaccagtatatatgattataactttttcctgtttccctatttccaaatggtcgaaaggaggaagttaggtctacctaagctgaatgtattcagttagcaggagaaatgaaatcctatacgtttaatactagaggagaaccgccttagaatatttatttcattggcaatgactccaggactacacagcgaaattgtattgcatgtgctgccaaaatactttagctctttccttcgaagtacgtcggatcctgtaattgagacaccgagtttaggtgactagggttttcttttgaggaggagtcccccaccccgccccgctctgccgcgacaggaagctagcgatccggaggacttagaatacaatcgtagtgtgggtaaacatggagggcaagcgcctgcaaagggaagtaagaagattcccagtccttgttgaaatccatttgcaaacagaggaagctgccgcgggtcgcagtcggtggggggaagccctgaaccccacgctgcacggctgggctggccaggtgcggccacgcccccatcgcggcggctggtaggagtgaatcagaccgtcagtattggtaaagaagtctgcggcagggcagggagggggaagagtagtcagtcgctcgctcactcgctcgctcgcacagacactgctgcagtgacactcggccctccagtgtcgcggagacgcaagagcagcgcgcagcacctgtccgcccggagcgagcccggcccgcggccgtagaaaaggagggaccgccgaggtgcgcgtcagtactgctcagcccggcagggacgcgggaggatgtggactgggtggac

SEQ ID NO: 32 - DNA, 2008 bp, Artificial Sequence
  recombinant or synthetic polynucleotide
gtggtgctgactcagcatcggttaataaaccctctgcaggaggctggatttcttttgtttaattatcacttggacctttctgagaactcttaagaattgttcattcgggtttttttgttttgttttggtttggtttttttgggttttttttttttttttttttttggtttttggagacagggtttctctgtatatagccctggcacaagagcaagctaacagcctgtttcttcttggtgctagcgccccctctggcagaaaatgaaataacaggtggacctacaacccccccccccccccccagtgtattctactcttgtccccggtataaatttgattgttccgaactacataaattgtagaaggattttttagatgcacatatcattttctgtgataccttccacacacccctcccccccaaaaaaatttttctgggaaagtttcttgaaaggaaaacagaagaacaagcctgtctttatgattgagttgggcttttgttttgctgtgtttcatttcttcctgtaaacaaatactcaaatgtccacttcattgtatgactaagttggtatcattaggttgggtctgggtgtgtgaatgtgggtgtggatctggatgtgggtgggtgtgtatgccccgtgtgtttagaatactagaaaagataccacatcgtaaacttttgggagagatgatttttaaaaatgggggtgggggtgaggggaacctgcgatgaggcaagcaagataaggggaagacttgagtttctgtgatctaaaaagtcgctgtgatgggatgctggctataaatgggcccttagcagcattgtttctgtgaattggaggatccctgctgaaggcaaaagaccattgaaggaagtaccgcatctggtttgttttgtaatgagaagcaggaatgcaaggtccacgctcttaataataaacaaacaggacattgtatgccatcatcacaggatgtccttccttctccagaagacagactggggctgaaggaaaagccggccaggctcagaacgagccccactaattactgcctccaacagctttccactcactgcccccagcccaacatcccctttttaactgggaagcattcctactctccattgtacgcacacgctcggaagcctggctgtgggtttgggcatgagaggcagggacaacaaaaccagtatatatgattataactttttcctgtttccctatttccaaatggtcgaaaggaggaagttaggtctacctaagctgaatgtattcagttagcaggagaaatgaaatcctatacgtttaatactagaggagaaccgccttagaatatttatttcattggcaatgactccaggactacacagcgaaattgtattgcatgtgctgccaaaatactttagctctttccttcgaagtacgtcggatcctgtaattgagacaccgagtttaggtgactagggttttcttttgaggaggagtcccccaccccgccccgctctgccgcgacaggaagctagcgatccggaggacttagaatacaatcgtagtgtgggtaaacatggagggcaagcgcctgcaaagggaagtaagaagattcccagtccttgttgaaatccatttgcaaacagaggaagctgccgcgggtcgcagtcggtggggggaagccctgaaccccacgctgcacggctgggctggccaggtgcggccacgcccccatcgcggcggctggtaggagtgaatcagaccgtcagtattggtaaagaagtctgcggcagggcagggagggggaagagtagtcagtcgctcgctcactcgctcgctcgcacagacactgctgcagtgacactcggccctccagtgtcgcggagacgcaagagcagcgcgcagcacctgtccgcccggagcgagcccggcccgcggccgtagaaaaggagggaccgccgaggtgcgcgtcagtactgctcagcccggcagggacgcgggaggatgtggactgggtggac

SEQ ID NO: 33 - DNA, 100 bp, Artificial Sequence
  recombinant or synthetic polynucleotide
gctctccacttcacttagatcttgctgtgaccaaggacaaggagaaaatgggtaccgatttaaatgatccagtggtcctgcagaggagagattgggagaa

SEQ ID NO: 34 - DNA, 100 bp, Artificial Sequence
  recombinant or synthetic polynucleotide
cagcccctagataacttcgtataatgtatgctatacgaagttatgctagcttccaggtgagtggctcaacgccctagcattcctccttccaactcttaat

SEQ ID NO: 35 - DNA, 172 bp, Artificial Sequence
  recombinant or synthetic polynucleotide
atcccccggctagagtttaaacactagaactagtggatccccgggctcgataactataacggtcctaaggtagcgactcgacataacttcgtataatgtatgctatacgaagttatgctagcttccaggtgagtggctcaacgccctagcattcctccttccaactcttaat

SEQ ID NO: 36 - DNA, 714 bp, Artificial Sequence
  recombinant or synthetic polynucleotide
ctggagtgtacctttgttgatagaacacttgtttaggattcgtgaaggtaaactgggcacccatctagaagcccagcactcagaggtggagacaggaggtcaggagttcaacaaggtcattctctgctacacagtgagtttaaaatcggcctgggatacacgagagagaccctgtgtaagagcagtagcagcagcaagaactcaagctgaaaaggaacatgcagtgtaagacaaagggccactgtgtgcatagagccagcaacctcacactgtaatgaacgggtctgacctttgcaagtaagcttcttgtgatgctctggttgagcctttgactacgacttttgtgacttgtgctcctctggatgcttgcaggatgagggtgaggacccctggtaccagaaagcatgcaagtgtgattgccaggtaggagccaatgctctgtggtctgctggagctacctccttagacagtattccaggtgagtggctcaacgccctagcattcctccttccaactcttaatccctctgctttctctcaagttggcttgtgagcttcacatctcaccgtggccactgctccaacattctgttcattatcaagtgccaggctctctccctccctggcttgcctgagatggtcaggtaagacccctcgagataacttcgtataatgtatgctatacgaagttatatgcatgccagtagcagcaccc

SEQ ID NO: 37 - DNA, 132 bp, Artificial Sequence
  recombinant or synthetic polynucleotide
ttccatcagacctcgacctgcagcccctagataacttcgtataatgtatgctatacgaagttatgctaggtaactataacggtcctaaggtagcgagctagcagcgtgagggaagtcccttcctcttaggta

SEQ ID NO: 38 - DNA, 760 bp, Artificial Sequence
  recombinant or synthetic polynucleotide
ctggagtgtacctttgttgatagaacacttgtttaggattcgtgaaggtaaactgggcacccatctagaagcccagcactcagaggtggagacaggaggtcaggagttcaacaaggtcattctctgctacacagtgagtttaaaatcggcctgggatacacgagagagaccctgtgtaagagcagtagcagcagcaagaactcaagctgaaaaggaacatgcagtgtaagacaaagggccactgtgtgcatagagccagcaacctcacactgtaatgaacgggtctgacctttgcaagtaagcttcttgtgatgctctggttgagcctttgactacgacttttgtgacttgtgctcctctggatgcttgcaggatgagggtgaggacccctggtaccagaaagcatgcaagtgtgattgccaggtaggagccaatgctctgtggtctgctggagctacctccttagacagtattccaggtgagtggctcaacgccctagcattcctccttccaactcttaatccctctgctttctctcaagttggcttgtgagcttcacatctcaccgtggccactgctccaacattctgttcattatcaagtgccaggctctctccctccctggcttgcctgagatggtcaggtaagacccctcgagataacttcgtataatgtatgctatacgaagttatgctaggtaactataacggtcctaaggtagcgagctagcagcgtgagggaagtcccttcctcttaggta

SEQ ID NO: 39 - DNA, 528 bp, Artificial Sequence
  recombinant or synthetic polynucleotide
tctttcctaaggaaaagaattaagagtcgggctatgtctgaaggcccagatacctcttgatgctaggtaacccttcaaaactcagcacctgttggctttttacagacatagataagaggatggctcctggtaatttggtgtgttcctggcaggtgtgcttggctttccaagtatcaggacagcagccagtggttacagatagatttgaaggagatcaaggtgatttcggggatcctgacccaaggatgctgtgacatagacgagtgggtgaccaagtacagtgtgcagtataggactgatgagcgcctgaactggatctactataaggatcagaccggaaacaatcgggtaagtgggggtcactccgagtcagcttcagctcacactgcggagacacactccatccctatgttcctgctgtccgcgtctgtctgagcattgacccctctacatgctgggtcatctgctcgagataacttcgtataatgtatgctatacgaagttatatgcatgccagtagcagcaccc

SEQ ID NO: 40 - DNA, 30 bp, Artificial Sequence
  recombinant or synthetic polynucleotide
ttttccagatgtgatctgggagactagcag

SEQ ID NO: 41 - DNA, 574 bp, Artificial Sequence
  recombinant or synthetic polynucleotide
tctttcctaaggaaaagaattaagagtcgggctatgtctgaaggcccagatacctcttgatgctaggtaacccttcaaaactcagcacctgttggctttttacagacatagataagaggatggctcctggtaatttggtgtgttcctggcaggtgtgcttggctttccaagtatcaggacagcagccagtggttacagatagatttgaaggagatcaaggtgatttcggggatcctgacccaaggatgctgtgacatagacgagtgggtgaccaagtacagtgtgcagtataggactgatgagcgcctgaactggatctactataaggatcagaccggaaacaatcgggtaagtgggggtcactccgagtcagcttcagctcacactgcggagacacactccatccctatgttcctgctgtccgcgtctgtctgagcattgacccctctacatgctgggtcatctgctcgagataacttcgtataatgtatgctatacgaagttatgctaggtaactataacggtcctaaggtagcgagctagcttttccagatgtgatctgggagactagcag

SEQ ID NO: 42 - DNA, 22 bp, Artificial Sequence
  synthetic oligonucleotide
tgggacaagtgtaaatgaggac

SEQ ID NO: 43 - DNA, 20 bp, Artificial Sequence
  synthetic oligonucleotide
agtggtgcttggccttatgc

SEQ ID NO: 44 - DNA, 26 bp, Artificial Sequence
  synthetic oligonucleotide
tcccaggcaaatcaggacaaagggtc

SEQ ID NO: 45 - DNA, 18 bp, Artificial Sequence
  synthetic oligonucleotide
gagccagcaacctcacac

SEQ ID NO: 46 - DNA, 21 bp, Artificial Sequence
  synthetic oligonucleotide
gcatccagaggagcacaagtc

SEQ ID NO: 47 - DNA, 27 bp, Artificial Sequence
  synthetic oligonucleotide
tgtaatgaacgggtctgacctttgcaa

SEQ ID NO: 48 - DNA, 24 bp, Artificial Sequence
  synthetic oligonucleotide
tcgtgaaggtcttgatttgatcct

SEQ ID NO: 49 - DNA, 20 bp, Artificial Sequence
  synthetic oligonucleotide
acctcctgtctccacctctg

SEQ ID NO: 50 - DNA, 24 bp, Artificial Sequence
  synthetic oligonucleotide
aagcaccatgtaaactgggcaccc

SEQ ID NO: 51 - DNA, 19 bp, Artificial Sequence
  synthetic oligonucleotide
ccctggcttgcctgagatg

SEQ ID NO: 52 - DNA, 21 bp, Artificial Sequence
  synthetic oligonucleotide
ggacttccctcacgctgagtt

SEQ ID NO: 53 - DNA, 26 bp, Artificial Sequence
  synthetic oligonucleotide
tcaggtaagacccaattgtcaatgca

SEQ ID NO: 54 - DNA, 21 bp, Artificial Sequence
  synthetic oligonucleotide
gagtcgggctatgtctgaagg

SEQ ID NO: 55 - DNA, 19 bp, Artificial Sequence
  synthetic oligonucleotide
gccaacaggtgctgagttt

SEQ ID NO: 56 - DNA, 28 bp, Artificial Sequence
  synthetic oligonucleotide
ccagatttgggatgatacctcttgatgc

SEQ ID NO: 57 - DNA, 22 bp, Artificial Sequence
  synthetic oligonucleotide
cctctacatgctgggtcatctg

SEQ ID NO: 58 - DNA, 21 bp, Artificial Sequence
  synthetic oligonucleotide
ggacttccctcacgctgagtt

SEQ ID NO: 59 - DNA, 24 bp, Artificial Sequence
  synthetic oligonucleotide
gacccacattcatttacaaactgc